European Patent Application EP 4 752 219 A2, published June 3, 2026. Title: RNA POLYMERASE VARIANT AND USE THEREOF. Applicant: Nanjing Novizan Biotechnology Co., Ltd. Application EP. The sequence listing filed with the application follows.

SEQUENCE LISTING (45 sequences)

SEQ ID NO: 1 - protein, 883 aa, synthetic construct
MNTINIAKNDFSDIELAAIPFNTLADHYGERLAREQLALEHESYEMGEARFRKMFERQLKAGEVADNAAAKPLITTLLPKMIARINDWFEEVKAKRGKRPTAFQFLQEIKPEAVAYITIKTTLACLTSADNTTVQAVASAIGRAIEDEARFGRIRDLEAKHFKKNVEEQLNKRVGHVYKKAFMQVVEADMLSKGLLGGEAWSSWHKEDSIHVGVRCIEMLIESTGMVSLHRQNAGVVGQDSETIELAPEYAEAIATRAGALAGISPMFQPCVVPPKPWTGITGGGYWANGRRPLALVRTHSKKALMRYEDVYMPEVYKAINIAQNTAWKINKKVLAVANVITKWKHCPVEDIPAIEREELPMKPEDIDMNPEALTAWKRAAAAVYRKDKARKSRRISLEFMLEQANKFANHKAIWFPYNMDWRGRVYAVSMFNPQGNDMTKGLLTLAKGKPIGKEGYYWLKIHGANCAGVDKVPFPERIKFIEENHENIMACAKSPLENTWWAEQDSPFCFLAFCFEYAGVQHHGLSYNCSLPLAFDGSCSGIQHFSAMLRDEVGGRAVNLLPSETVQDIYGIVAKKVNEILQADAINGTDNEVVTVTDENTGEISEKVKLGTKALAGQWLAYGVTRSVTKRSVMTLAYGSKEFGFRQQVLEDTIQPAIDSGKGLMFTQPNQAAGYMAKLIWESVSVTVVAAVEAMNWLKSAAKLLAAEVKDKKTGEILRKRCAVHWVTPDGFPVWQEYKKPIQTRLNLMFLGQFRLQPTINTNKDSEIDAHKQESGIAPNFVHSQDGSHLRKTVVWAHEKYGIESFALIHDSFGTIPADAANLFKAVRETMVDTYESCDVLADFYDQFADQLHESQLDKMPALPAKGNLNLRDILESDFAFA

SEQ ID NO: 2 - protein, 883 aa, synthetic construct
MNTINIAKNDFSDIELAAIPFNTLADHYGERLAREQLALEHESYEMGEARFRKMFERQLKAGEVADNAAAKPLITTLLPKMIARINDWFEEVKAKRGKRPTAFQFLQEIKPEAVAYITIKTTLACLTSADNTTVQAVASAIGRAIEDEARFGRIRDLEAKHFKKNVEEQLNKRVGHVYKKAFMQVVEADMLSKGLLGGEAWSSWHKEDSIHVGVRCIEMLIESTGMVSLHRQNAGVVGQDSETIELAPEYAEAIATRAGALAGISPMFQPCVVPPKPWTGITGGGYWANGRRPLALVRTHSKKALMRYEDVYMPEVYKAINIAQNTAWKINKKVLAVANVITKWKHCPVEDIPAIEREELPMKPEDIDMNPEALTAWKRAAAAVYCKDKARKSRRISLEFMLEQANKFANHKAIWFPYNMDWRGRVYAVSMFNPQGNDMTKGLLTLAKGKPIGKEGYYWLKIHGANCAGVDKVPFPERIKFIEENHENIMACAKSPLENTWWAEQDSPFCFLAFCFEYAGVQHHGLSYNCSLPLAFDGSCSGIQHFSAMLRDEVGGRAVNLLPSETVQDIYGIVAKKVNEILQADAINGTDNEVVTVTDENTGEISEKVKLGTKALAGQWLAYGVTRSVTKRSVMTLAYGSKEFGFRQQVLEDTIQPAIDSGKGLMFTQPNQAAGYMAKLIWESVSVTVVAAVEAMNWLKSAAKLLAAEVKDKKTGEILRKRCAVHWVTPDGFPVWQEYKKPIQTRLNLMFLGQFRLQPTINTNKDSEIDAHKQESGIAPNFVHSQDGSHLRKTVVWAHEKYGIESFALIHDSFGTIPADAANLFKAVRETMVDTYESCDVLADFYDQFADQLHESQLDKMPALPAKGNLNLRDILESDFAFA

SEQ ID NO: 3 - protein, 883 aa, synthetic construct
MNTINIAKNDFSDIELAAIPFNTLADHYGERLAREQLALEHESYEMGEARFRKMFERQLKAGEVADNAAAKPLITTLLPKMIARINDWFEEVKAKRGKRPTAFQFLQEIKPEAVAYITIKTTLACLTSADNTTVQAVASAIGRAIEDEARFGRIRDLEAKHFKKNVEEQLNKRVGHVYKKAFMQVVEADMLSKGLLGGEAWSSWHKEDSIHVGVRCIEMLIESTGMVSLHRQNAGVVGQDSETIELAPEYAEAIATRAGALAGISPMFQPCVVPPKPWTGITGGGYWANGRRPLALVRTHSKKALMRYEDVYMPEVYKAINIAQNTAWKINKKVLAVANVITKWKHCPVEDIPAIEREELPMKPEDIDMNPEALTAWKRAAAAVYWKDKARKSRRISLEFMLEQANKFANHKAIWFPYNMDWRGRVYAVSMFNPQGNDMTKGLLTLAKGKPIGKEGYYWLKIHGANCAGVDKVPFPERIKFIEENHENIMACAKSPLENTWWAEQDSPFCFLAFCFEYAGVQHHGLSYNCSLPLAFDGSCSGIQHFSAMLRDEVGGRAVNLLPSETVQDIYGIVAKKVNEILQADAINGTDNEVVTVTDENTGEISEKVKLGTKALAGQWLAYGVTRSVTKRSVMTLAYGSKEFGFRQQVLEDTIQPAIDSGKGLMFTQPNQAAGYMAKLIWESVSVTVVAAVEAMNWLKSAAKLLAAEVKDKKTGEILRKRCAVHWVTPDGFPVWQEYKKPIQTRLNLMFLGQFRLQPTINTNKDSEIDAHKQESGIAPNFVHSQDGSHLRKTVVWAHEKYGIESFALIHDSFGTIPADAANLFKAVRETMVDTYESCDVLADFYDQFADQLHESQLDKMPALPAKGNLNLRDILESDFAFA

SEQ ID NO: 4 - protein, 883 aa, synthetic construct
MNTINIAKNDFSDIELAAIPFNTLADHYGERLAREQLALEHESYEMGEARFRKMFERQLKAGEVADNAAAKPLITTLLPKMIARINDWFEEVKAKRGKRPTAFQFLQEIKPEAVAYITIKTTLACLTSADNTTVQAVASAIGRAIEDEARFGRIRDLEAKHFKKNVEEQLNKRVGHVYKKAFMQVVEADMLSKGLLGGEAWSSWHKEDSIHVGVRCIEMLIESTGMVSLHRQNAGVVGQDSETIELAPEYAEAIATRAGALAGISPMFQPCVVPPKPWTGITGGGYWANGRRPLALVRTHSKKALMRYEDVYMPEVYKAINIAQNTAWKINKKVLAVANVITKWKHCPVEDIPAIEREELPMKPEDIDMNPEALTAWKRAAAAVYRKKKARKSRRISLEFMLEQANKFANHKAIWFPYNMDWRGRVYAVSMFNPQGNDMTKGLLTLAKGKPIGKEGYYWLKIHGANCAGVDKVPFPERIKFIEENHENIMACAKSPLENTWWAEQDSPFCFLAFCFEYAGVQHHGLSYNCSLPLAFDGSCSGIQHFSAMLRDEVGGRAVNLLPSETVQDIYGIVAKKVNEILQADAINGTDNEVVTVTDENTGEISEKVKLGTKALAGQWLAYGVTRSVTKRSVMTLAYGSKEFGFRQQVLEDTIQPAIDSGKGLMFTQPNQAAGYMAKLIWESVSVTVVAAVEAMNWLKSAAKLLAAEVKDKKTGEILRKRCAVHWVTPDGFPVWQEYKKPIQTRLNLMFLGQFRLQPTINTNKDSEIDAHKQESGIAPNFVHSQDGSHLRKTVVWAHEKYGIESFALIHDSFGTIPADAANLFKAVRETMVDTYESCDVLADFYDQFADQLHESQLDKMPALPAKGNLNLRDILESDFAFA

SEQ ID NO: 5 - protein, 883 aa, synthetic construct
MNTINIAKNDFSDIELAAIPFNTLADHYGERLAREQLALEHESYEMGEARFRKMFERQLKAGEVADNAAAKPLITTLLPKMIARINDWFEEVKAKRGKRPTAFQFLQEIKPEAVAYITIKTTLACLTSADNTTVQAVASAIGRAIEDEARFGRIRDLEAKHFKKNVEEQLNKRVGHVYKKAFMQVVEADMLSKGLLGGEAWSSWHKEDSIHVGVRCIEMLIESTGMVSLHRQNAGVVGQDSETIELAPEYAEAIATRAGALAGISPMFQPCVVPPKPWTGITGGGYWANGRRPLALVRTHSKKALMRYEDVYMPEVYKAINIAQNTAWKINKKVLAVANVITKWKHCPVEDIPAIEREELPMKPEDIDMNPEALTAWKRAAAAVYRKDKARKSRRISLEFMLEQANKFANHKAIWFPYNMDWRGRVYAVSMFNPAGNDMTKGLLTLAKGKPIGKEGYYWLKIHGANCAGVDKVPFPERIKFIEENHENIMACAKSPLENTWWAEQDSPFCFLAFCFEYAGVQHHGLSYNCSLPLAFDGSCSGIQHFSAMLRDEVGGRAVNLLPSETVQDIYGIVAKKVNEILQADAINGTDNEVVTVTDENTGEISEKVKLGTKALAGQWLAYGVTRSVTKRSVMTLAYGSKEFGFRQQVLEDTIQPAIDSGKGLMFTQPNQAAGYMAKLIWESVSVTVVAAVEAMNWLKSAAKLLAAEVKDKKTGEILRKRCAVHWVTPDGFPVWQEYKKPIQTRLNLMFLGQFRLQPTINTNKDSEIDAHKQESGIAPNFVHSQDGSHLRKTVVWAHEKYGIESFALIHDSFGTIPADAANLFKAVRETMVDTYESCDVLADFYDQFADQLHESQLDKMPALPAKGNLNLRDILESDFAFA

SEQ ID NO: 6 - protein, 883 aa, synthetic construct
MNTINIAKNDFSDIELAAIPFNTLADHYGERLAREQLALEHESYEMGEARFRKMFERQLKAGEVADNAAAKPLITTLLPKMIARINDWFEEVKAKRGKRPTAFQFLQEIKPEAVAYITIKTTLACLTSADNTTVQAVASAIGRAIEDEARFGRIRDLEAKHFKKNVEEQLNKRVGHVYKKAFMQVVEADMLSKGLLGGEAWSSWHKEDSIHVGVRCIEMLIESTGMVSLHRQNAGVVGQDSETIELAPEYAEAIATRAGALAGISPMFQPCVVPPKPWTGITGGGYWANGRRPLALVRTHSKKALMRYEDVYMPEVYKAINIAQNTAWKINKKVLAVANVITKWKHCPVEDIPAIEREELPMKPEDIDMNPEALTAWKRAAAAVYRKDKARKSRRISLEFMLEQANKFANHKAIWFPYNMDWRGRVYAVSMFNPHGNDMTKGLLTLAKGKPIGKEGYYWLKIHGANCAGVDKVPFPERIKFIEENHENIMACAKSPLENTWWAEQDSPFCFLAFCFEYAGVQHHGLSYNCSLPLAFDGSCSGIQHFSAMLRDEVGGRAVNLLPSETVQDIYGIVAKKVNEILQADAINGTDNEVVTVTDENTGEISEKVKLGTKALAGQWLAYGVTRSVTKRSVMTLAYGSKEFGFRQQVLEDTIQPAIDSGKGLMFTQPNQAAGYMAKLIWESVSVTVVAAVEAMNWLKSAAKLLAAEVKDKKTGEILRKRCAVHWVTPDGFPVWQEYKKPIQTRLNLMFLGQFRLQPTINTNKDSEIDAHKQESGIAPNFVHSQDGSHLRKTVVWAHEKYGIESFALIHDSFGTIPADAANLFKAVRETMVDTYESCDVLADFYDQFADQLHESQLDKMPALPAKGNLNLRDILESDFAFA

SEQ ID NO: 7 - protein, 883 aa, synthetic construct
MNTINIAKNDFSDIELAAIPFNTLADHYGERLAREQLALEHESYEMGEARFRKMFERQLKAGEVADNAAAKPLITTLLPKMIARINDWFEEVKAKRGKRPTAFQFLQEIKPEAVAYITIKTTLACLTSADNTTVQAVASAIGRAIEDEARFGRIRDLEAKHFKKNVEEQLNKRVGHVYKKAFMQVVEADMLSKGLLGGEAWSSWHKEDSIHVGVRCIEMLIESTGMVSLHRQNAGVVGQDSETIELAPEYAEAIATRAGALAGISPMFQPCVVPPKPWTGITGGGYWANGRRPLALVRTHSKKALMRYEDVYMPEVYKAINIAQNTAWKINKKVLAVANVITKWKHCPVEDIPAIEREELPMKPEDIDMNPEALTAWKRAAAAVYRKDKARKSRRISLEFMLEQANKFANHKAIWFPYNMDWRGRVYAVSMFNPTGNDMTKGLLTLAKGKPIGKEGYYWLKIHGANCAGVDKVPFPERIKFIEENHENIMACAKSPLENTWWAEQDSPFCFLAFCFEYAGVQHHGLSYNCSLPLAFDGSCSGIQHFSAMLRDEVGGRAVNLLPSETVQDIYGIVAKKVNEILQADAINGTDNEVVTVTDENTGEISEKVKLGTKALAGQWLAYGVTRSVTKRSVMTLAYGSKEFGFRQQVLEDTIQPAIDSGKGLMFTQPNQAAGYMAKLIWESVSVTVVAAVEAMNWLKSAAKLLAAEVKDKKTGEILRKRCAVHWVTPDGFPVWQEYKKPIQTRLNLMFLGQFRLQPTINTNKDSEIDAHKQESGIAPNFVHSQDGSHLRKTVVWAHEKYGIESFALIHDSFGTIPADAANLFKAVRETMVDTYESCDVLADFYDQFADQLHESQLDKMPALPAKGNLNLRDILESDFAFA

SEQ ID NO: 8 - protein, 883 aa, synthetic construct
MNTINIAKNDFSDIELAAIPFNTLADHYGERLAREQLALEHESYEMGEARFRKMFERQLKAGEVADNAAAKPLITTLLPKMIARINDWFEEVKAKRGKRPTAFQFLQEIKPEAVAYITIKTTLACLTSADNTTVQAVASAIGRAIEDEARFGRIRDLEAKHFKKNVEEQLNKRVGHVYKKAFMQVVEADMLSKGLLGGEAWSSWHKEDSIHVGVRCIEMLIESTGMVSLHRQNAGVVGQDSETIELAPEYAEAIATRAGALAGISPMFQPCVVPPKPWTGITGGGYWANGRRPLALVRTHSKKALMRYEDVYMPEVYKAINIAQNTAWKINKKVLAVANVITKWKHCPVEDIPAIEREELPMKPEDIDMNPEALTAWKRAAAAVYRKDKARKSRRISLEFMLEQANKFANHKAIWFPYNMDWRGRVYAVSMFNPQGFDMTKGLLTLAKGKPIGKEGYYWLKIHGANCAGVDKVPFPERIKFIEENHENIMACAKSPLENTWWAEQDSPFCFLAFCFEYAGVQHHGLSYNCSLPLAFDGSCSGIQHFSAMLRDEVGGRAVNLLPSETVQDIYGIVAKKVNEILQADAINGTDNEVVTVTDENTGEISEKVKLGTKALAGQWLAYGVTRSVTKRSVMTLAYGSKEFGFRQQVLEDTIQPAIDSGKGLMFTQPNQAAGYMAKLIWESVSVTVVAAVEAMNWLKSAAKLLAAEVKDKKTGEILRKRCAVHWVTPDGFPVWQEYKKPIQTRLNLMFLGQFRLQPTINTNKDSEIDAHKQESGIAPNFVHSQDGSHLRKTVVWAHEKYGIESFALIHDSFGTIPADAANLFKAVRETMVDTYESCDVLADFYDQFADQLHESQLDKMPALPAKGNLNLRDILESDFAFA

SEQ ID NO: 9 - protein, 883 aa, synthetic construct
MNTINIAKNDFSDIELAAIPFNTLADHYGERLAREQLALEHESYEMGEARFRKMFERQLKAGEVADNAAAKPLITTLLPKMIARINDWFEEVKAKRGKRPTAFQFLQEIKPEAVAYITIKTTLACLTSADNTTVQAVASAIGRAIEDEARFGRIRDLEAKHFKKNVEEQLNKRVGHVYKKAFMQVVEADMLSKGLLGGEAWSSWHKEDSIHVGVRCIEMLIESTGMVSLHRQNAGVVGQDSETIELAPEYAEAIATRAGALAGISPMFQPCVVPPKPWTGITGGGYWANGRRPLALVRTHSKKALMRYEDVYMPEVYKAINIAQNTAWKINKKVLAVANVITKWKHCPVEDIPAIEREELPMKPEDIDMNPEALTAWKRAAAAVYRKDKARKSRRISLEFMLEQANKFANHKAIWFPYNMDWRGRVYAVSMFNPQGTDMTKGLLTLAKGKPIGKEGYYWLKIHGANCAGVDKVPFPERIKFIEENHENIMACAKSPLENTWWAEQDSPFCFLAFCFEYAGVQHHGLSYNCSLPLAFDGSCSGIQHFSAMLRDEVGGRAVNLLPSETVQDIYGIVAKKVNEILQADAINGTDNEVVTVTDENTGEISEKVKLGTKALAGQWLAYGVTRSVTKRSVMTLAYGSKEFGFRQQVLEDTIQPAIDSGKGLMFTQPNQAAGYMAKLIWESVSVTVVAAVEAMNWLKSAAKLLAAEVKDKKTGEILRKRCAVHWVTPDGFPVWQEYKKPIQTRLNLMFLGQFRLQPTINTNKDSEIDAHKQESGIAPNFVHSQDGSHLRKTVVWAHEKYGIESFALIHDSFGTIPADAANLFKAVRETMVDTYESCDVLADFYDQFADQLHESQLDKMPALPAKGNLNLRDILESDFAFA

SEQ ID NO: 10 - protein, 883 aa, synthetic construct
MNTINIAKNDFSDIELAAIPFNTLADHYGERLAREQLALEHESYEMGEARFRKMFERQLKAGEVADNAAAKPLITTLLPKMIARINDWFEEVKAKRGKRPTAFQFLQEIKPEAVAYITIKTTLACLTSADNTTVQAVASAIGRAIEDEARFGRIRDLEAKHFKKNVEEQLNKRVGHVYKKAFMQVVEADMLSKGLLGGEAWSSWHKEDSIHVGVRCIEMLIESTGMVSLHRQNAGVVGQDSETIELAPEYAEAIATRAGALAGISPMFQPCVVPPKPWTGITGGGYWANGRRPLALVRTHSKKALMRYEDVYMPEVYKAINIAQNTAWKINKKVLAVANVITKWKHCPVEDIPAIEREELPMKPEDIDMNPEALTAWKRAAAAVYRKDKARKSRRISLEFMLEQANKFANHKAIWFPYNMDWRGRVYAVSMFNPQGNTMTKGLLTLAKGKPIGKEGYYWLKIHGANCAGVDKVPFPERIKFIEENHENIMACAKSPLENTWWAEQDSPFCFLAFCFEYAGVQHHGLSYNCSLPLAFDGSCSGIQHFSAMLRDEVGGRAVNLLPSETVQDIYGIVAKKVNEILQADAINGTDNEVVTVTDENTGEISEKVKLGTKALAGQWLAYGVTRSVTKRSVMTLAYGSKEFGFRQQVLEDTIQPAIDSGKGLMFTQPNQAAGYMAKLIWESVSVTVVAAVEAMNWLKSAAKLLAAEVKDKKTGEILRKRCAVHWVTPDGFPVWQEYKKPIQTRLNLMFLGQFRLQPTINTNKDSEIDAHKQESGIAPNFVHSQDGSHLRKTVVWAHEKYGIESFALIHDSFGTIPADAANLFKAVRETMVDTYESCDVLADFYDQFADQLHESQLDKMPALPAKGNLNLRDILESDFAFA

SEQ ID NO: 11 - protein, 883 aa, synthetic construct
MNTINIAKNDFSDIELAAIPFNTLADHYGERLAREQLALEHESYEMGEARFRKMFERQLKAGEVADNAAAKPLITTLLPKMIARINDWFEEVKAKRGKRPTAFQFLQEIKPEAVAYITIKTTLACLTSADNTTVQAVASAIGRAIEDEARFGRIRDLEAKHFKKNVEEQLNKRVGHVYKKAFMQVVEADMLSKGLLGGEAWSSWHKEDSIHVGVRCIEMLIESTGMVSLHRQNAGVVGQDSETIELAPEYAEAIATRAGALAGISPMFQPCVVPPKPWTGITGGGYWANGRRPLALVRTHSKKALMRYEDVYMPEVYKAINIAQNTAWKINKKVLAVANVITKWKHCPVEDIPAIEREELPMKPEDIDMNPEALTAWKRAAAAVYRKDKARKSRRISLEFMLEQANKFANHKAIWFPYNMDWRGRVYAVSMFNPQGNLMTKGLLTLAKGKPIGKEGYYWLKIHGANCAGVDKVPFPERIKFIEENHENIMACAKSPLENTWWAEQDSPFCFLAFCFEYAGVQHHGLSYNCSLPLAFDGSCSGIQHFSAMLRDEVGGRAVNLLPSETVQDIYGIVAKKVNEILQADAINGTDNEVVTVTDENTGEISEKVKLGTKALAGQWLAYGVTRSVTKRSVMTLAYGSKEFGFRQQVLEDTIQPAIDSGKGLMFTQPNQAAGYMAKLIWESVSVTVVAAVEAMNWLKSAAKLLAAEVKDKKTGEILRKRCAVHWVTPDGFPVWQEYKKPIQTRLNLMFLGQFRLQPTINTNKDSEIDAHKQESGIAPNFVHSQDGSHLRKTVVWAHEKYGIESFALIHDSFGTIPADAANLFKAVRETMVDTYESCDVLADFYDQFADQLHESQLDKMPALPAKGNLNLRDILESDFAFA

SEQ ID NO: 12 - protein, 883 aa, synthetic construct
MNTINIAKNDFSDIELAAIPFNTLADHYGERLAREQLALEHESYEMGEARFRKMFERQLKAGEVADNAAAKPLITTLLPKMIARINDWFEEVKAKRGKRPTAFQFLQEIKPEAVAYITIKTTLACLTSADNTTVQAVASAIGRAIEDEARFGRIRDLEAKHFKKNVEEQLNKRVGHVYKKAFMQVVEADMLSKGLLGGEAWSSWHKEDSIHVGVRCIEMLIESTGMVSLHRQNAGVVGQDSETIELAPEYAEAIATRAGALAGISPMFQPCVVPPKPWTGITGGGYWANGRRPLALVRTHSKKALMRYEDVYMPEVYKAINIAQNTAWKINKKVLAVANVITKWKHCPVEDIPAIEREELPMKPEDIDMNPEALTAWKRAAAAVYRKDKARKSRRISLEFMLEQANKFANHKAIWFPYNMDWRGRVYAVSMFNPQGNIMTKGLLTLAKGKPIGKEGYYWLKIHGANCAGVDKVPFPERIKFIEENHENIMACAKSPLENTWWAEQDSPFCFLAFCFEYAGVQHHGLSYNCSLPLAFDGSCSGIQHFSAMLRDEVGGRAVNLLPSETVQDIYGIVAKKVNEILQADAINGTDNEVVTVTDENTGEISEKVKLGTKALAGQWLAYGVTRSVTKRSVMTLAYGSKEFGFRQQVLEDTIQPAIDSGKGLMFTQPNQAAGYMAKLIWESVSVTVVAAVEAMNWLKSAAKLLAAEVKDKKTGEILRKRCAVHWVTPDGFPVWQEYKKPIQTRLNLMFLGQFRLQPTINTNKDSEIDAHKQESGIAPNFVHSQDGSHLRKTVVWAHEKYGIESFALIHDSFGTIPADAANLFKAVRETMVDTYESCDVLADFYDQFADQLHESQLDKMPALPAKGNLNLRDILESDFAFA

SEQ ID NO: 13 - protein, 883 aa, synthetic construct
MNTINIAKNDFSDIELAAIPFNTLADHYGERLAREQLALEHESYEMGEARFRKMFERQLKAGEVADNAAAKPLITTLLPKMIARINDWFEEVKAKRGKRPTAFQFLQEIKPEAVAYITIKTTLACLTSADNTTVQAVASAIGRAIEDEARFGRIRDLEAKHFKKNVEEQLNKRVGHVYKKAFMQVVEADMLSKGLLGGEAWSSWHKEDSIHVGVRCIEMLIESTGMVSLHRQNAGVVGQDSETIELAPEYAEAIATRAGALAGISPMFQPCVVPPKPWTGITGGGYWANGRRPLALVRTHSKKALMRYEDVYMPEVYKAINIAQNTAWKINKKVLAVANVITKWKHCPVEDIPAIEREELPMKPEDIDMNPEALTAWKRAAAAVYRKDKARKSRRISLEFMLEQANKFANHKAIWFPYNMDWRGRVYAVSMFNPQGNPMTKGLLTLAKGKPIGKEGYYWLKIHGANCAGVDKVPFPERIKFIEENHENIMACAKSPLENTWWAEQDSPFCFLAFCFEYAGVQHHGLSYNCSLPLAFDGSCSGIQHFSAMLRDEVGGRAVNLLPSETVQDIYGIVAKKVNEILQADAINGTDNEVVTVTDENTGEISEKVKLGTKALAGQWLAYGVTRSVTKRSVMTLAYGSKEFGFRQQVLEDTIQPAIDSGKGLMFTQPNQAAGYMAKLIWESVSVTVVAAVEAMNWLKSAAKLLAAEVKDKKTGEILRKRCAVHWVTPDGFPVWQEYKKPIQTRLNLMFLGQFRLQPTINTNKDSEIDAHKQESGIAPNFVHSQDGSHLRKTVVWAHEKYGIESFALIHDSFGTIPADAANLFKAVRETMVDTYESCDVLADFYDQFADQLHESQLDKMPALPAKGNLNLRDILESDFAFA

SEQ ID NO: 14 - protein, 883 aa, synthetic construct
MNTINIAKNDFSDIELAAIPFNTLADHYGERLAREQLALEHESYEMGEARFRKMFERQLKAGEVADNAAAKPLITTLLPKMIARINDWFEEVKAKRGKRPTAFQFLQEIKPEAVAYITIKTTLACLTSADNTTVQAVASAIGRAIEDEARFGRIRDLEAKHFKKNVEEQLNKRVGHVYKKAFMQVVEADMLSKGLLGGEAWSSWHKEDSIHVGVRCIEMLIESTGMVSLHRQNAGVVGQDSETIELAPEYAEAIATRAGALAGISPMFQPCVVPPKPWTGITGGGYWANGRRPLALVRTHSKKALMRYEDVYMPEVYKAINIAQNTAWKINKKVLAVANVITKWKHCPVEDIPAIEREELPMKPEDIDMNPEALTAWKRAAAAVYRKDKARKSRRISLEFMLEQANKFANHKAIWFPYNMDWRGRVYAVSMFNPQGNVMTKGLLTLAKGKPIGKEGYYWLKIHGANCAGVDKVPFPERIKFIEENHENIMACAKSPLENTWWAEQDSPFCFLAFCFEYAGVQHHGLSYNCSLPLAFDGSCSGIQHFSAMLRDEVGGRAVNLLPSETVQDIYGIVAKKVNEILQADAINGTDNEVVTVTDENTGEISEKVKLGTKALAGQWLAYGVTRSVTKRSVMTLAYGSKEFGFRQQVLEDTIQPAIDSGKGLMFTQPNQAAGYMAKLIWESVSVTVVAAVEAMNWLKSAAKLLAAEVKDKKTGEILRKRCAVHWVTPDGFPVWQEYKKPIQTRLNLMFLGQFRLQPTINTNKDSEIDAHKQESGIAPNFVHSQDGSHLRKTVVWAHEKYGIESFALIHDSFGTIPADAANLFKAVRETMVDTYESCDVLADFYDQFADQLHESQLDKMPALPAKGNLNLRDILESDFAFA

SEQ ID NO: 15 - protein, 883 aa, synthetic construct
MNTINIAKNDFSDIELAAIPFNTLADHYGERLAAEQLALEHESYEMGEARFRKMFERQLKAGEVADNAAAKPLITTLLPKMIARINDWFEEVKAKRGKRPTAFQFLQEIKPEAVAYITIKTTLACLTSADNTTVQAVASAIGRAIEDEARFGRIRDLEAKHFKKNVEEQLNKRVGHVYKKAFMQVVEADMLSKGLLGGEAWSSWHKEDSIHVGVRCIEMLIESTGMVSLHRQNAGVVGQDSETIELAPEYAEAIATRAGALAGISPMFQPCVVPPKPWTGITGGGYWANGRRPLALVRTHSKKALMRYEDVYMPEVYKAINIAQNTAWKINKKVLAVANVITKWKHCPVEDIPAIEREELPMKPEDIDMNPEALTAWKRAAAAVYAKDKARKSRRISLEFMLEQANKFANHKAIWFPYNMDWRGRVYAVSMFNPQGNDMTKGLLTLAKGKPIGKEGYYWLKIHGANCAGVDKVPFPERIKFIEENHENIMACAKSPLENTWWAEQDSPFCFLAFCFEYAGVQHHGLSYNCSLPLAFDGSCSGIQHFSAMLRDEVGGRAVNLLPSETVQDIYGIVAKKVNEILQADAINGTDNEVVTVTDENTGEISEKVKLGTKALAGQWLAYGVTRSVTKRSVMTLAYGSKEFGFRQQVLEDTIQPAIDSGKGLMFTQPNQAAGYMAKLIWESVSVTVVAAVEAMNWLKSAAKLLAAEVKDKKTGEILRKRCAVHWVTPDGFPVWQEYKKPIQTRLNLMFLGQFRLQPTINTNKDSEIDAHKQESGIAPNFVHSQDGSHLRKTVVWAHEKYGIESFALIHDSFGTIPADAANLFKAVRETMVDTYESCDVLADFYDQFADQLHESQLDKMPALPAKGNLNLRDILESDFAFA

SEQ ID NO: 16 - protein, 883 aa, synthetic construct
MNTINIAKNDFSDIELAAIPFNTLADHYGERLAAEQLALEHESYEMGEARFRKMFERQLKAGEVADNAAAKPLITTLLPKMIARINDWFEEVKAKRGKRPTAFQFLQEIKPEAVAYITIKTTLACLTSADNTTVQAVASAIGRAIEDEARFGRIRDLEAKHFKKNVEEQLNKRVGHVYKKAFMQVVEADMLSKGLLGGEAWSSWHKEDSIHVGVRCIEMLIESTGMVSLHRQNAGVVGQDSETIELAPEYAEAIATRAGALAGISPMFQPCVVPPKPWTGITGGGYWANGRRPLALVRTHSKKALMRYEDVYMPEVYKAINIAQNTAWKINKKVLAVANVITKWKHCPVEDIPAIEREELPMKPEDIDMNPEALTAWKRAAAAVYMKDKARKSRRISLEFMLEQANKFANHKAIWFPYNMDWRGRVYAVSMFNPQGNDMTKGLLTLAKGKPIGKEGYYWLKIHGANCAGVDKVPFPERIKFIEENHENIMACAKSPLENTWWAEQDSPFCFLAFCFEYAGVQHHGLSYNCSLPLAFDGSCSGIQHFSAMLRDEVGGRAVNLLPSETVQDIYGIVAKKVNEILQADAINGTDNEVVTVTDENTGEISEKVKLGTKALAGQWLAYGVTRSVTKRSVMTLAYGSKEFGFRQQVLEDTIQPAIDSGKGLMFTQPNQAAGYMAKLIWESVSVTVVAAVEAMNWLKSAAKLLAAEVKDKKTGEILRKRCAVHWVTPDGFPVWQEYKKPIQTRLNLMFLGQFRLQPTINTNKDSEIDAHKQESGIAPNFVHSQDGSHLRKTVVWAHEKYGIESFALIHDSFGTIPADAANLFKAVRETMVDTYESCDVLADFYDQFADQLHESQLDKMPALPAKGNLNLRDILESDFAFA

SEQ ID NO: 17 - protein, 883 aa, synthetic construct
MNTINIAKNDFSDIELAAIPFNTLADHYGERLAREQLALEHESYEMGEARFRKMFERQLKAGEVADNAAAKPLITTLLPKMIARINDWFEEVKAKRGKRPTAFQFLQEIKPEAVAYITIKTTLACLTSADNTTVQAVASAIGRAIEDEARFGRIRDLEAKHFKKNVEEQLNKRVGHVHKKAFMQVVEADMLSKGLLGGEAWSSWHKEDSIHVGVRCIEMLIESTGMVSLHRQNAGVVGQDSETIELAPEYAEAIATRAGALAGISPMFQPCVVPPKPWTGITGGGYWANGRRPLALVRTHSKKALMRYEDVYMPEVYKAINIAQNTAWKINKKVLAVANVITKWKHCPVEDIPAIEREELPMKPEDIDMNPEALTAWKRAAAAVYMKDKARKSRRISLEFMLEQANKFANHKAIWFPYNMDWRGRVYAVSMFNPQGNDMTKGLLTLAKGKPIGKEGYYWLKIHGANCAGVDKVPFPERIKFIEENHENIMACAKSPLENTWWAEQDSPFCFLAFCFEYAGVQHHGLSYNCSLPLAFDGSCSGIQHFSAMLRDEVGGRAVNLLPSETVQDIYGIVAKKVNEILQADAINGTDNEVVTVTDENTGEISEKVKLGTKALAGQWLAYGVTRSVTKRSVMTLAYGSKEFGFRQQVLEDTIQPAIDSGKGLMFTQPNQAAGYMAKLIWESVSVTVVAAVEAMNWLKSAAKLLAAEVKDKKTGEILRKRCAVHWVTPDGFPVWQEYKKPIQTRLNLMFLGQFRLQPTINTNKDSEIDAHKQESGIAPNFVHSQDGSHLRKTVVWAHEKYGIESFALIHDSFGTIPADAANLFKAVRETMVDTYESCDVLADFYDQFADQLHESQLDKMPALPAKGNLNLRDILESDFAFA

SEQ ID NO: 18 - protein, 883 aa, synthetic construct
MNTINIAKNDFSDIELAAIPFNTLADHYGERLAREQLALEHESYEMGEARFRKMFERQLKAGEVADNAAAKPLITTLLPKMIARINDWFEEVKAKRGKRPTAFQFLQEIKPEAVAYITIKTTLACLTSADNTTVQAVASAIGRAIEDEARFGRIRDLEAKHFKKNVEEQLNKRVGHVYKKAFMQVVEADMLSKGLLGGEAWSSWHKEDSIHVGVRCIEMLIESTGMVSLHRQNAGVVGQDSETIELAPEYAEAIATRAGALAGISPMFQPCVVPPKPWTGITGGGYWANGRRPLALVRTHSKKALMRYEDVYMPEVYKAINIAQNTAWKINKKVLAVANVITKWKHCPVEDIPAIEREELPMKPEDIDMNPEALTAWKRAAAAVYWKDKARKSRRISLEFMLEQANKFANHKAIWFPYNMDWRGRVYAVSMFNPQGTDMTKGLLTLAKGKPIGKEGYYWLKIHGANCAGVDKVPFPERIKFIEENHENIMACAKSPLENTWWAEQDSPFCFLAFCFEYAGVQHHGLSYNCSLPLAFDGSCSGIQHFSAMLRDEVGGRAVNLLPSETVQDIYGIVAKKVNEILQADAINGTDNEVVTVTDENTGEISEKVKLGTKALAGQWLAYGVTRSVTKRSVMTLAYGSKEFGFRQQVLEDTIQPAIDSGKGLMFTQPNQAAGYMAKLIWESVSVTVVAAVEAMNWLKSAAKLLAAEVKDKKTGEILRKRCAVHWVTPDGFPVWQEYKKPIQTRLNLMFLGQFRLQPTINTNKDSEIDAHKQESGIAPNFVHSQDGSHLRKTVVWAHEKYGIESFALIHDSFGTIPADAANLFKAVRETMVDTYESCDVLADFYDQFADQLHESQLDKMPALPAKGNLNLRDILESDFAFA

SEQ ID NO: 19 - protein, 882 aa, synthetic construct
MNTINIAKNDFSDIELAAIPFNTLADHYGERLAREQLALEHESYEMGEARFRKMFERQLKAGEVADNAAAKPLITTLLPKMIARINDWFEEVKAKRGKRPTAFQFLQEIKPEAVAYITIKTTLACLTSADNTTVQAVASAIGRAIEDEARFGRIRDLEAKHFKKNVEEQLNRVGHVYKKAFMQVVEADMLSKGLLGGEAWSSWHKEDSIHVGVRCIEMLIESTGMVSLHRQNAGVVGQDSETIELAPEYAEAIATRAGALAGISPMFQPCVVPPKPWTGITGGGYWANGRRPLALVRTHSKKALMRYEDVYMPEVYKAINIAQNTAWKINKKVLAVANVITKWKHCPVEDIPAIEREELPMKPEDIDMNPEALTAWKRAAAAVYIKDKARKSRRISLEFMLEQANKFANHKAIWFPYNMDWRGRVYAVSMFNPQGNDMTKGLLTLAKGKPIGKEGYYWLKIHGANCAGVDKVPFPERIKFIEENHENIMACAKSPLENTWWAEQDSPFCFLAFCFEYAGVQHHGLSYNCSLPLAFDGSCSGIQHFSAMLRDEVGGRAVNLLPSETVQDIYGIVAKKVNEILQADAINGTDNEVVTVTDENTGEISEKVKLGTKALAGQWLAYGVTRSVTKRSVMTLAYGSKEFGFRQQVLEDTIQPAIDSGKGLMFTQPNQAAGYMAKLIWESVSVTVVAAVEAMNWLKSAAKLLAAEVKDKKTGEILRKRCAVHWVTPDGFPVWQEYKKPIQTRLNLMFLGQFRLQPTINTNKDSEIDAHKQESGIAPNFVHSQDGSHLRKTVVWAHEKYGIESFALIHDSFGTIPADAANLFKAVRETMVDTYESCDVLADFYDQFADQLHESQLDKMPALPAKGNLNLRDILESDFAFA

SEQ ID NO: 20 - protein, 883 aa, synthetic construct
MNTINIAKNDFSDIELAAIPFNTLADHYGERLAREQLALEHESYEMGEARFRKMFERQLKAGEVADNAAAKPLITTLLPKMIARINDWFEEVKAKRGKRPTAFQFLQEIKPEAVAYITIKTTLACLTSADNTTVQAVASAIGRAIEDEARFGRIRDLEAKHFKKNVEEQLNKRVGHVDKKAFMQVVEADMLSKGLLGGEAWSSWHKEDSIHVGVRCIEMLIESTGMVSLHRQNAGVVGQDSETIELAPEYAEAIATRAGALAGISPMFQPCVVPPKPWTGITGGGYWANGRRPLALVRTHSKKALMRYEDVYMPEVYKAINIAQNTAWKINKKVLAVANVITKWKHCPVEDIPAIEREELPMKPEDIDMNPEALTAWKRAAAAVYFKDKARKSRRISLEFMLEQANKFANHKAIWFPYNMDWRGRVYAVSMFNPQGNDMTKGLLTLAKGKPIGKEGYYWLKIHGANCAGVDKVPFPERIKFIEENHENIMACAKSPLENTWWAEQDSPFCFLAFCFEYAGVQHHGLSYNCSLPLAFDGSCSGIQHFSAMLRDEVGGRAVNLLPSETVQDIYGIVAKKVNEILQADAINGTDNEVVTVTDENTGEISEKVKLGTKALAGQWLAYGVTRSVTKRSVMTLAYGSKEFGFRQQVLEDTIQPAIDSGKGLMFTQPNQAAGYMAKLIWESVSVTVVAAVEAMNWLKSAAKLLAAEVKDKKTGEILRKRCAVHWVTPDGFPVWQEYKKPIQTRLNLMFLGQFRLQPTINTNKDSEIDAHKQESGIAPNFVHSQDGSHLRKTVVWAHEKYGIESFALIHDSFGTIPADAANLFKAVRETMVDTYESCDVLADFYDQFADQLHESQLDKMPALPAKGNLNLRDILESDFAFA

SEQ ID NO: 21 - protein, 883 aa, synthetic construct
MNTINIAKNDFSDIELAAIPFNTLADHYGERLAREQLALEHESYEMGEARFRKMFERQLKAGEVADNAAAKPLITTLLPKMIARINDWFEEVKAKRGKRPTAFQFLQEIKPEAVAYITIKTTLACLTSADNTTVQAVASAIGRAIEDEARFGRIRDLEAKHFKKNVEEQLNKRVGHVYKKAFMQVVEADMLSKGLLGGEAWSSWHKEDSIHVGVRCIEMLIESTGMVSLHRQNAGVVGQDSETIELAPEYAEAIATRAGALAGISPMFQPCVVPPKPWTGITGGGYWANGRRPLALVRTHSKKALMRYEDVYMPEVYKAINIAQNTAWKINKKVLAVANVITKWKHCPVEDIPAIEREELPMKPEDIDMNPEALTAWKRAAAAVYRKKKARKSRRISLEFMLEQANKFANHKAIWFPYNMDWRGRVYAVSMFNPQGNPMTKGLLTLAKGKPIGKEGYYWLKIHGANCAGVDKVPFPERIKFIEENHENIMACAKSPLENTWWAEQDSPFCFLAFCFEYAGVQHHGLSYNCSLPLAFDGSCSGIQHFSAMLRDEVGGRAVNLLPSETVQDIYGIVAKKVNEILQADAINGTDNEVVTVTDENTGEISEKVKLGTKALAGQWLAYGVTRSVTKRSVMTLAYGSKEFGFRQQVLEDTIQPAIDSGKGLMFTQPNQAAGYMAKLIWESVSVTVVAAVEAMNWLKSAAKLLAAEVKDKKTGEILRKRCAVHWVTPDGFPVWQEYKKPIQTRLNLMFLGQFRLQPTINTNKDSEIDAHKQESGIAPNFVHSQDGSHLRKTVVWAHEKYGIESFALIHDSFGTIPADAANLFKAVRETMVDTYESCDVLADFYDQFADQLHESQLDKMPALPAKGNLNLRDILESDFAFA

SEQ ID NO: 22 - protein, 883 aa, synthetic construct
MNTINIAKNDFSDIELAAIPFNTLADHYGERLAREQLALEHESYEMGEARFRKMFERQLKAGEVADNAAAKPLITTLLPKMIARINDWFEEVKAKRGKRPTAFQFLQEIKPEAVAYITIKTTLACLTSADNTTVQAVASAIGRAIEDEARFGRIRDLEAKHFKKNVEEQLNKRVGHVYKKAFMQVVEADMLSKGLLGGEAWSSWHKEDSIHVGVRCIEMLIESTGMVSLHRQNAGVVGQDSETIELAPEYAEAIATRAGALAGISPMFQPCVVPPKPWTGITGGGYWANGRRPLALVRTHSKKALMRYEDVYMPEVYKAINIAQNTAWKINKKVLAVANVITKWKHCPVEDIPAIEREELPMKPEDIDMNPEALTAWKRAAAAVYCKDKARKSRRISLEFMLEQANKFANHKAIWFPYNMDWRGRVYAVSMFNPQGNPMTKGLLTLAKGKPIGKEGYYWLKIHGANCAGVDKVPFPERIKFIEENHENIMACAKSPLENTWWAEQDSPFCFLAFCFEYAGVQHHGLSYNCSLPLAFDGSCSGIQHFSAMLRDEVGGRAVNLLPSETVQDIYGIVAKKVNEILQADAINGTDNEVVTVTDENTGEISEKVKLGTKALAGQWLAYGVTRSVTKRSVMTLAYGSKEFGFRQQVLEDTIQPAIDSGKGLMFTQPNQAAGYMAKLIWESVSVTVVAAVEAMNWLKSAAKLLAAEVKDKKTGEILRKRCAVHWVTPDGFPVWQEYKKPIQTRLNLMFLGQFRLQPTINTNKDSEIDAHKQESGIAPNFVHSQDGSHLRKTVVWAHEKYGIESFALIHDSFGTIPADAANLFKAVRETMVDTYESCDVLADFYDQFADQLHESQLDKMPALPAKGNLNLRDILESDFAFA

SEQ ID NO: 23 - DNA, 2652 bp, synthetic construct
  source 1..2652: mol_type = other DNA
atgaatacaattaacatagctaaaaatgatttcagcgatattgaactggctgcgatcccgtttaataccttggcggaccattatggtgagcgtctggcgcgtgagcaacttgctctggagcacgaatcctacgagatgggtgaagcgcgtttccggaagatgttcgagcgccagcttaaggctggcgaggtggcggataacgctgctgcgaagccgttgattacgaccctgctgccgaaaatgattgcgcgtattaacgattggttcgaggaagtgaaagcaaagcgtggtaaacgtccaaccgcattccagtttctgcaagagatcaagccggaggcggtggcatacattacgatcaaaaccactctcgcatgtctcaccagcgcggataatactacggtccaagcggtggccagcgcgattggccgcgcgattgaggacgaagcgcgttttggtcgcattcgtgacctggaagcgaaacattttaagaagaacgttgaagaacaattgaataaacgcgtgggccacgtttacaagaaagcgttcatgcaagtcgttgaagctgatatgctgagcaaaggcctgttaggtggtgaagcatggagcagctggcataaggaggactcaattcacgtcggcgtgcggtgcattgaaatgctgatcgaatcgaccggtatggttagcctgcatcgccaaaacgccggcgtggtgggtcaagatagcgaaacgattgaactggcgccagagtacgcggaagctatcgctaccagagccggcgcattggcggggatcagcccgatgttccagccgtgtgttgtaccaccgaagccgtggaccggtatcaccggtggaggttactgggcgaatggtagacgtccgttggcgttggttcgtacccatagcaaaaaggctctgatgcgttatgaagacgtttacatgccggaagtgtacaaagccatcaacatcgcgcagaacactgcgtggaaaatcaacaaaaaggtgttagctgtggcgaacgtaattacaaaatggaagcactgcccggttgaggacatcccggctattgaacgtgaagagctgccaatgaaaccagaggacattgacatgaatccggaggcgctgaccgcatggaaacgtgcggcagcagcggtctatcgtaaggataaagccagaaagagccgtcgtatctccctggaattcatgcttgagcaggcgaacaaattcgctaaccacaaagccatctggtttccgtataatatggattggcgtggtcgtgtttacgcggtatcgatgttcaacccgcagggtaatgacatgaccaagggtttgttgaccttggccaaaggtaaaccgattggcaaagaaggttactattggttgaagatccacggtgcgaactgcgcaggggtggataaggtaccgttcccggaacgtattaaattcatcgaggaaaaccacgaaaacattatggcgtgcgcaaagagcccgctggaaaacacgtggtgggcagagcaggacagtccattctgcttcttggcgttctgtttcgaatatgcaggtgtccagcaccacggcctgagctataactgcagcctgccgctggcctttgatggttcttgtagcggtattcaacactttagcgccatgctgcgcgatgaggttggtggcagagcagtgaatctgctgccaagcgaaaccgtgcaagatatctatggcattgtggctaagaaggttaatgaaatcctgcaagcagacgcgattaacggcacggacaacgaggttgtcaccgtgaccgatgaaaacaccggtgagatctcggagaaagtgaaactgggcaccaaagccttggctggccaatggctggcatacggcgttactcgctccgtgaccaagcgttcggtgatgacccttgcttacggcagcaaagagtttggtttccgccaacaggttctggaggatactatccaaccggccatcgactctggtaaaggcctgatgttcacgcagccgaatcaggcagcgggctatatggcgaagctgatttgggaatcggttagcgttaccgttgttgcagcggtggaggctatgaactggctgaaatctgcggcgaagctgttagctgcggaggtgaaggacaagaagacgggcgaaatcctgcgtaagcgctgcgcagtgcattgggttacgccggatggttttccggtatggcaggagtacaaaaagcctattcagacccgtctgaacctgatgtttctgggtcaatttcgtctgcagccgacgatcaacaccaataaggactccgagatcgacgcgcacaaacaggagtctggcatcgcacccaatttcgttcactcacaggacggttcccatctgcgtaagaccgtcgtgtgggcacacgagaagtatggcattgagtcgtttgcattgatccacgattcctttggtaccatcccggcggacgctgcgaacctgtttaaagcggttcgcgaaaccatggttgacacctatgaaagttgcgatgttctggcagacttttatgatcagttcgccgaccaactgcatgagtcccagctggataaaatgccggcgttaccggcgaagggcaacttaaatctccgcgacatcctggaatctgatttcgccttcgcgtaa

SEQ ID NO: 24 - DNA, 2652 bp, synthetic construct
  source 1..2652: mol_type = other DNA
atgaatacaattaacatagctaaaaatgatttcagcgatattgaactggctgcgatcccgtttaataccttggcggaccattatggtgagcgtctggcgcgtgagcaacttgctctggagcacgaatcctacgagatgggtgaagcgcgtttccggaagatgttcgagcgccagcttaaggctggcgaggtggcggataacgctgctgcgaagccgttgattacgaccctgctgccgaaaatgattgcgcgtattaacgattggttcgaggaagtgaaagcaaagcgtggtaaacgtccaaccgcattccagtttctgcaagagatcaagccggaggcggtggcatacattacgatcaaaaccactctcgcatgtctcaccagcgcggataatactacggtccaagcggtggccagcgcgattggccgcgcgattgaggacgaagcgcgttttggtcgcattcgtgacctggaagcgaaacattttaagaagaacgttgaagaacaattgaataaacgcgtgggccacgtttacaagaaagcgttcatgcaagtcgttgaagctgatatgctgagcaaaggcctgttaggtggtgaagcatggagcagctggcataaggaggactcaattcacgtcggcgtgcggtgcattgaaatgctgatcgaatcgaccggtatggttagcctgcatcgccaaaacgccggcgtggtgggtcaagatagcgaaacgattgaactggcgccagagtacgcggaagctatcgctaccagagccggcgcattggcggggatcagcccgatgttccagccgtgtgttgtaccaccgaagccgtggaccggtatcaccggtggaggttactgggcgaatggtagacgtccgttggcgttggttcgtacccatagcaaaaaggctctgatgcgttatgaagacgtttacatgccggaagtgtacaaagccatcaacatcgcgcagaacactgcgtggaaaatcaacaaaaaggtgttagctgtggcgaacgtaattacaaaatggaagcactgcccggttgaggacatcccggctattgaacgtgaagagctgccaatgaaaccagaggacattgacatgaatccggaggcgctgaccgcatggaaacgtgcggcagcagcggtctattgcaaggataaagccagaaagagccgtcgtatctccctggaattcatgcttgagcaggcgaacaaattcgctaaccacaaagccatctggtttccgtataatatggattggcgtggtcgtgtttacgcggtatcgatgttcaacccgcagggtaatgacatgaccaagggtttgttgaccttggccaaaggtaaaccgattggcaaagaaggttactattggttgaagatccacggtgcgaactgcgcaggggtggataaggtaccgttcccggaacgtattaaattcatcgaggaaaaccacgaaaacattatggcgtgcgcaaagagcccgctggaaaacacgtggtgggcagagcaggacagtccattctgcttcttggcgttctgtttcgaatatgcaggtgtccagcaccacggcctgagctataactgcagcctgccgctggcctttgatggttcttgtagcggtattcaacactttagcgccatgctgcgcgatgaggttggtggcagagcagtgaatctgctgccaagcgaaaccgtgcaagatatctatggcattgtggctaagaaggttaatgaaatcctgcaagcagacgcgattaacggcacggacaacgaggttgtcaccgtgaccgatgaaaacaccggtgagatctcggagaaagtgaaactgggcaccaaagccttggctggccaatggctggcatacggcgttactcgctccgtgaccaagcgttcggtgatgacccttgcttacggcagcaaagagtttggtttccgccaacaggttctggaggatactatccaaccggccatcgactctggtaaaggcctgatgttcacgcagccgaatcaggcagcgggctatatggcgaagctgatttgggaatcggttagcgttaccgttgttgcagcggtggaggctatgaactggctgaaatctgcggcgaagctgttagctgcggaggtgaaggacaagaagacgggcgaaatcctgcgtaagcgctgcgcagtgcattgggttacgccggatggttttccggtatggcaggagtacaaaaagcctattcagacccgtctgaacctgatgtttctgggtcaatttcgtctgcagccgacgatcaacaccaataaggactccgagatcgacgcgcacaaacaggagtctggcatcgcacccaatttcgttcactcacaggacggttcccatctgcgtaagaccgtcgtgtgggcacacgagaagtatggcattgagtcgtttgcattgatccacgattcctttggtaccatcccggcggacgctgcgaacctgtttaaagcggttcgcgaaaccatggttgacacctatgaaagttgcgatgttctggcagacttttatgatcagttcgccgaccaactgcatgagtcccagctggataaaatgccggcgttaccggcgaagggcaacttaaatctccgcgacatcctggaatctgatttcgccttcgcgtaa

SEQ ID NO: 25 - DNA, 2652 bp, synthetic construct
  source 1..2652: mol_type = other DNA
atgaatacaattaacatagctaaaaatgatttcagcgatattgaactggctgcgatcccgtttaataccttggcggaccattatggtgagcgtctggcgcgtgagcaacttgctctggagcacgaatcctacgagatgggtgaagcgcgtttccggaagatgttcgagcgccagcttaaggctggcgaggtggcggataacgctgctgcgaagccgttgattacgaccctgctgccgaaaatgattgcgcgtattaacgattggttcgaggaagtgaaagcaaagcgtggtaaacgtccaaccgcattccagtttctgcaagagatcaagccggaggcggtggcatacattacgatcaaaaccactctcgcatgtctcaccagcgcggataatactacggtccaagcggtggccagcgcgattggccgcgcgattgaggacgaagcgcgttttggtcgcattcgtgacctggaagcgaaacattttaagaagaacgttgaagaacaattgaataaacgcgtgggccacgtttacaagaaagcgttcatgcaagtcgttgaagctgatatgctgagcaaaggcctgttaggtggtgaagcatggagcagctggcataaggaggactcaattcacgtcggcgtgcggtgcattgaaatgctgatcgaatcgaccggtatggttagcctgcatcgccaaaacgccggcgtggtgggtcaagatagcgaaacgattgaactggcgccagagtacgcggaagctatcgctaccagagccggcgcattggcggggatcagcccgatgttccagccgtgtgttgtaccaccgaagccgtggaccggtatcaccggtggaggttactgggcgaatggtagacgtccgttggcgttggttcgtacccatagcaaaaaggctctgatgcgttatgaagacgtttacatgccggaagtgtacaaagccatcaacatcgcgcagaacactgcgtggaaaatcaacaaaaaggtgttagctgtggcgaacgtaattacaaaatggaagcactgcccggttgaggacatcccggctattgaacgtgaagagctgccaatgaaaccagaggacattgacatgaatccggaggcgctgaccgcatggaaacgtgcggcagcagcggtctattggaaggataaagccagaaagagccgtcgtatctccctggaattcatgcttgagcaggcgaacaaattcgctaaccacaaagccatctggtttccgtataatatggattggcgtggtcgtgtttacgcggtatcgatgttcaacccgcagggtaatgacatgaccaagggtttgttgaccttggccaaaggtaaaccgattggcaaagaaggttactattggttgaagatccacggtgcgaactgcgcaggggtggataaggtaccgttcccggaacgtattaaattcatcgaggaaaaccacgaaaacattatggcgtgcgcaaagagcccgctggaaaacacgtggtgggcagagcaggacagtccattctgcttcttggcgttctgtttcgaatatgcaggtgtccagcaccacggcctgagctataactgcagcctgccgctggcctttgatggttcttgtagcggtattcaacactttagcgccatgctgcgcgatgaggttggtggcagagcagtgaatctgctgccaagcgaaaccgtgcaagatatctatggcattgtggctaagaaggttaatgaaatcctgcaagcagacgcgattaacggcacggacaacgaggttgtcaccgtgaccgatgaaaacaccggtgagatctcggagaaagtgaaactgggcaccaaagccttggctggccaatggctggcatacggcgttactcgctccgtgaccaagcgttcggtgatgacccttgcttacggcagcaaagagtttggtttccgccaacaggttctggaggatactatccaaccggccatcgactctggtaaaggcctgatgttcacgcagccgaatcaggcagcgggctatatggcgaagctgatttgggaatcggttagcgttaccgttgttgcagcggtggaggctatgaactggctgaaatctgcggcgaagctgttagctgcggaggtgaaggacaagaagacgggcgaaatcctgcgtaagcgctgcgcagtgcattgggttacgccggatggttttccggtatggcaggagtacaaaaagcctattcagacccgtctgaacctgatgtttctgggtcaatttcgtctgcagccgacgatcaacaccaataaggactccgagatcgacgcgcacaaacaggagtctggcatcgcacccaatttcgttcactcacaggacggttcccatctgcgtaagaccgtcgtgtgggcacacgagaagtatggcattgagtcgtttgcattgatccacgattcctttggtaccatcccggcggacgctgcgaacctgtttaaagcggttcgcgaaaccatggttgacacctatgaaagttgcgatgttctggcagacttttatgatcagttcgccgaccaactgcatgagtcccagctggataaaatgccggcgttaccggcgaagggcaacttaaatctccgcgacatcctggaatctgatttcgccttcgcgtaa

SEQ ID NO: 26 - DNA, 2652 bp, synthetic construct
  source 1..2652: mol_type = other DNA
atgaatacaattaacatagctaaaaatgatttcagcgatattgaactggctgcgatcccgtttaataccttggcggaccattatggtgagcgtctggcgcgtgagcaacttgctctggagcacgaatcctacgagatgggtgaagcgcgtttccggaagatgttcgagcgccagcttaaggctggcgaggtggcggataacgctgctgcgaagccgttgattacgaccctgctgccgaaaatgattgcgcgtattaacgattggttcgaggaagtgaaagcaaagcgtggtaaacgtccaaccgcattccagtttctgcaagagatcaagccggaggcggtggcatacattacgatcaaaaccactctcgcatgtctcaccagcgcggataatactacggtccaagcggtggccagcgcgattggccgcgcgattgaggacgaagcgcgttttggtcgcattcgtgacctggaagcgaaacattttaagaagaacgttgaagaacaattgaataaacgcgtgggccacgtttacaagaaagcgttcatgcaagtcgttgaagctgatatgctgagcaaaggcctgttaggtggtgaagcatggagcagctggcataaggaggactcaattcacgtcggcgtgcggtgcattgaaatgctgatcgaatcgaccggtatggttagcctgcatcgccaaaacgccggcgtggtgggtcaagatagcgaaacgattgaactggcgccagagtacgcggaagctatcgctaccagagccggcgcattggcggggatcagcccgatgttccagccgtgtgttgtaccaccgaagccgtggaccggtatcaccggtggaggttactgggcgaatggtagacgtccgttggcgttggttcgtacccatagcaaaaaggctctgatgcgttatgaagacgtttacatgccggaagtgtacaaagccatcaacatcgcgcagaacactgcgtggaaaatcaacaaaaaggtgttagctgtggcgaacgtaattacaaaatggaagcactgcccggttgaggacatcccggctattgaacgtgaagagctgccaatgaaaccagaggacattgacatgaatccggaggcgctgaccgcatggaaacgtgcggcagcagcggtctatcgtaagaaaaaagccagaaagagccgtcgtatctccctggaattcatgcttgagcaggcgaacaaattcgctaaccacaaagccatctggtttccgtataatatggattggcgtggtcgtgtttacgcggtatcgatgttcaacccgcagggtaatgacatgaccaagggtttgttgaccttggccaaaggtaaaccgattggcaaagaaggttactattggttgaagatccacggtgcgaactgcgcaggggtggataaggtaccgttcccggaacgtattaaattcatcgaggaaaaccacgaaaacattatggcgtgcgcaaagagcccgctggaaaacacgtggtgggcagagcaggacagtccattctgcttcttggcgttctgtttcgaatatgcaggtgtccagcaccacggcctgagctataactgcagcctgccgctggcctttgatggttcttgtagcggtattcaacactttagcgccatgctgcgcgatgaggttggtggcagagcagtgaatctgctgccaagcgaaaccgtgcaagatatctatggcattgtggctaagaaggttaatgaaatcctgcaagcagacgcgattaacggcacggacaacgaggttgtcaccgtgaccgatgaaaacaccggtgagatctcggagaaagtgaaactgggcaccaaagccttggctggccaatggctggcatacggcgttactcgctccgtgaccaagcgttcggtgatgacccttgcttacggcagcaaagagtttggtttccgccaacaggttctggaggatactatccaaccggccatcgactctggtaaaggcctgatgttcacgcagccgaatcaggcagcgggctatatggcgaagctgatttgggaatcggttagcgttaccgttgttgcagcggtggaggctatgaactggctgaaatctgcggcgaagctgttagctgcggaggtgaaggacaagaagacgggcgaaatcctgcgtaagcgctgcgcagtgcattgggttacgccggatggttttccggtatggcaggagtacaaaaagcctattcagacccgtctgaacctgatgtttctgggtcaatttcgtctgcagccgacgatcaacaccaataaggactccgagatcgacgcgcacaaacaggagtctggcatcgcacccaatttcgttcactcacaggacggttcccatctgcgtaagaccgtcgtgtgggcacacgagaagtatggcattgagtcgtttgcattgatccacgattcctttggtaccatcccggcggacgctgcgaacctgtttaaagcggttcgcgaaaccatggttgacacctatgaaagttgcgatgttctggcagacttttatgatcagttcgccgaccaactgcatgagtcccagctggataaaatgccggcgttaccggcgaagggcaacttaaatctccgcgacatcctggaatctgatttcgccttcgcgtaa

SEQ ID NO: 27 - DNA, 2652 bp, synthetic construct
  source 1..2652: mol_type = other DNA
atgaatacaattaacatagctaaaaatgatttcagcgatattgaactggctgcgatcccgtttaataccttggcggaccattatggtgagcgtctggcgcgtgagcaacttgctctggagcacgaatcctacgagatgggtgaagcgcgtttccggaagatgttcgagcgccagcttaaggctggcgaggtggcggataacgctgctgcgaagccgttgattacgaccctgctgccgaaaatgattgcgcgtattaacgattggttcgaggaagtgaaagcaaagcgtggtaaacgtccaaccgcattccagtttctgcaagagatcaagccggaggcggtggcatacattacgatcaaaaccactctcgcatgtctcaccagcgcggataatactacggtccaagcggtggccagcgcgattggccgcgcgattgaggacgaagcgcgttttggtcgcattcgtgacctggaagcgaaacattttaagaagaacgttgaagaacaattgaataaacgcgtgggccacgtttacaagaaagcgttcatgcaagtcgttgaagctgatatgctgagcaaaggcctgttaggtggtgaagcatggagcagctggcataaggaggactcaattcacgtcggcgtgcggtgcattgaaatgctgatcgaatcgaccggtatggttagcctgcatcgccaaaacgccggcgtggtgggtcaagatagcgaaacgattgaactggcgccagagtacgcggaagctatcgctaccagagccggcgcattggcggggatcagcccgatgttccagccgtgtgttgtaccaccgaagccgtggaccggtatcaccggtggaggttactgggcgaatggtagacgtccgttggcgttggttcgtacccatagcaaaaaggctctgatgcgttatgaagacgtttacatgccggaagtgtacaaagccatcaacatcgcgcagaacactgcgtggaaaatcaacaaaaaggtgttagctgtggcgaacgtaattacaaaatggaagcactgcccggttgaggacatcccggctattgaacgtgaagagctgccaatgaaaccagaggacattgacatgaatccggaggcgctgaccgcatggaaacgtgcggcagcagcggtctatcgtaaggataaagccagaaagagccgtcgtatctccctggaattcatgcttgagcaggcgaacaaattcgctaaccacaaagccatctggtttccgtataatatggattggcgtggtcgtgtttacgcggtatcgatgttcaacccggctggtaatgacatgaccaagggtttgttgaccttggccaaaggtaaaccgattggcaaagaaggttactattggttgaagatccacggtgcgaactgcgcaggggtggataaggtaccgttcccggaacgtattaaattcatcgaggaaaaccacgaaaacattatggcgtgcgcaaagagcccgctggaaaacacgtggtgggcagagcaggacagtccattctgcttcttggcgttctgtttcgaatatgcaggtgtccagcaccacggcctgagctataactgcagcctgccgctggcctttgatggttcttgtagcggtattcaacactttagcgccatgctgcgcgatgaggttggtggcagagcagtgaatctgctgccaagcgaaaccgtgcaagatatctatggcattgtggctaagaaggttaatgaaatcctgcaagcagacgcgattaacggcacggacaacgaggttgtcaccgtgaccgatgaaaacaccggtgagatctcggagaaagtgaaactgggcaccaaagccttggctggccaatggctggcatacggcgttactcgctccgtgaccaagcgttcggtgatgacccttgcttacggcagcaaagagtttggtttccgccaacaggttctggaggatactatccaaccggccatcgactctggtaaaggcctgatgttcacgcagccgaatcaggcagcgggctatatggcgaagctgatttgggaatcggttagcgttaccgttgttgcagcggtggaggctatgaactggctgaaatctgcggcgaagctgttagctgcggaggtgaaggacaagaagacgggcgaaatcctgcgtaagcgctgcgcagtgcattgggttacgccggatggttttccggtatggcaggagtacaaaaagcctattcagacccgtctgaacctgatgtttctgggtcaatttcgtctgcagccgacgatcaacaccaataaggactccgagatcgacgcgcacaaacaggagtctggcatcgcacccaatttcgttcactcacaggacggttcccatctgcgtaagaccgtcgtgtgggcacacgagaagtatggcattgagtcgtttgcattgatccacgattcctttggtaccatcccggcggacgctgcgaacctgtttaaagcggttcgcgaaaccatggttgacacctatgaaagttgcgatgttctggcagacttttatgatcagttcgccgaccaactgcatgagtcccagctggataaaatgccggcgttaccggcgaagggcaacttaaatctccgcgacatcctggaatctgatttcgccttcgcgtaa

SEQ ID NO: 28 - DNA, 2652 bp, synthetic construct
  source 1..2652: mol_type = other DNA
atgaatacaattaacatagctaaaaatgatttcagcgatattgaactggctgcgatcccgtttaataccttggcggaccattatggtgagcgtctggcgcgtgagcaacttgctctggagcacgaatcctacgagatgggtgaagcgcgtttccggaagatgttcgagcgccagcttaaggctggcgaggtggcggataacgctgctgcgaagccgttgattacgaccctgctgccgaaaatgattgcgcgtattaacgattggttcgaggaagtgaaagcaaagcgtggtaaacgtccaaccgcattccagtttctgcaagagatcaagccggaggcggtggcatacattacgatcaaaaccactctcgcatgtctcaccagcgcggataatactacggtccaagcggtggccagcgcgattggccgcgcgattgaggacgaagcgcgttttggtcgcattcgtgacctggaagcgaaacattttaagaagaacgttgaagaacaattgaataaacgcgtgggccacgtttacaagaaagcgttcatgcaagtcgttgaagctgatatgctgagcaaaggcctgttaggtggtgaagcatggagcagctggcataaggaggactcaattcacgtcggcgtgcggtgcattgaaatgctgatcgaatcgaccggtatggttagcctgcatcgccaaaacgccggcgtggtgggtcaagatagcgaaacgattgaactggcgccagagtacgcggaagctatcgctaccagagccggcgcattggcggggatcagcccgatgttccagccgtgtgttgtaccaccgaagccgtggaccggtatcaccggtggaggttactgggcgaatggtagacgtccgttggcgttggttcgtacccatagcaaaaaggctctgatgcgttatgaagacgtttacatgccggaagtgtacaaagccatcaacatcgcgcagaacactgcgtggaaaatcaacaaaaaggtgttagctgtggcgaacgtaattacaaaatggaagcactgcccggttgaggacatcccggctattgaacgtgaagagctgccaatgaaaccagaggacattgacatgaatccggaggcgctgaccgcatggaaacgtgcggcagcagcggtctatcgtaaggataaagccagaaagagccgtcgtatctccctggaattcatgcttgagcaggcgaacaaattcgctaaccacaaagccatctggtttccgtataatatggattggcgtggtcgtgtttacgcggtatcgatgttcaacccgcatggtaatgacatgaccaagggtttgttgaccttggccaaaggtaaaccgattggcaaagaaggttactattggttgaagatccacggtgcgaactgcgcaggggtggataaggtaccgttcccggaacgtattaaattcatcgaggaaaaccacgaaaacattatggcgtgcgcaaagagcccgctggaaaacacgtggtgggcagagcaggacagtccattctgcttcttggcgttctgtttcgaatatgcaggtgtccagcaccacggcctgagctataactgcagcctgccgctggcctttgatggttcttgtagcggtattcaacactttagcgccatgctgcgcgatgaggttggtggcagagcagtgaatctgctgccaagcgaaaccgtgcaagatatctatggcattgtggctaagaaggttaatgaaatcctgcaagcagacgcgattaacggcacggacaacgaggttgtcaccgtgaccgatgaaaacaccggtgagatctcggagaaagtgaaactgggcaccaaagccttggctggccaatggctggcatacggcgttactcgctccgtgaccaagcgttcggtgatgacccttgcttacggcagcaaagagtttggtttccgccaacaggttctggaggatactatccaaccggccatcgactctggtaaaggcctgatgttcacgcagccgaatcaggcagcgggctatatggcgaagctgatttgggaatcggttagcgttaccgttgttgcagcggtggaggctatgaactggctgaaatctgcggcgaagctgttagctgcggaggtgaaggacaagaagacgggcgaaatcctgcgtaagcgctgcgcagtgcattgggttacgccggatggttttccggtatggcaggagtacaaaaagcctattcagacccgtctgaacctgatgtttctgggtcaatttcgtctgcagccgacgatcaacaccaataaggactccgagatcgacgcgcacaaacaggagtctggcatcgcacccaatttcgttcactcacaggacggttcccatctgcgtaagaccgtcgtgtgggcacacgagaagtatggcattgagtcgtttgcattgatccacgattcctttggtaccatcccggcggacgctgcgaacctgtttaaagcggttcgcgaaaccatggttgacacctatgaaagttgcgatgttctggcagacttttatgatcagttcgccgaccaactgcatgagtcccagctggataaaatgccggcgttaccggcgaagggcaacttaaatctccgcgacatcctggaatctgatttcgccttcgcgtaa

SEQ ID NO: 29 - DNA, 2652 bp, synthetic construct
  source 1..2652: mol_type = other DNA
atgaatacaattaacatagctaaaaatgatttcagcgatattgaactggctgcgatcccgtttaataccttggcggaccattatggtgagcgtctggcgcgtgagcaacttgctctggagcacgaatcctacgagatgggtgaagcgcgtttccggaagatgttcgagcgccagcttaaggctggcgaggtggcggataacgctgctgcgaagccgttgattacgaccctgctgccgaaaatgattgcgcgtattaacgattggttcgaggaagtgaaagcaaagcgtggtaaacgtccaaccgcattccagtttctgcaagagatcaagccggaggcggtggcatacattacgatcaaaaccactctcgcatgtctcaccagcgcggataatactacggtccaagcggtggccagcgcgattggccgcgcgattgaggacgaagcgcgttttggtcgcattcgtgacctggaagcgaaacattttaagaagaacgttgaagaacaattgaataaacgcgtgggccacgtttacaagaaagcgttcatgcaagtcgttgaagctgatatgctgagcaaaggcctgttaggtggtgaagcatggagcagctggcataaggaggactcaattcacgtcggcgtgcggtgcattgaaatgctgatcgaatcgaccggtatggttagcctgcatcgccaaaacgccggcgtggtgggtcaagatagcgaaacgattgaactggcgccagagtacgcggaagctatcgctaccagagccggcgcattggcggggatcagcccgatgttccagccgtgtgttgtaccaccgaagccgtggaccggtatcaccggtggaggttactgggcgaatggtagacgtccgttggcgttggttcgtacccatagcaaaaaggctctgatgcgttatgaagacgtttacatgccggaagtgtacaaagccatcaacatcgcgcagaacactgcgtggaaaatcaacaaaaaggtgttagctgtggcgaacgtaattacaaaatggaagcactgcccggttgaggacatcccggctattgaacgtgaagagctgccaatgaaaccagaggacattgacatgaatccggaggcgctgaccgcatggaaacgtgcggcagcagcggtctatcgtaaggataaagccagaaagagccgtcgtatctccctggaattcatgcttgagcaggcgaacaaattcgctaaccacaaagccatctggtttccgtataatatggattggcgtggtcgtgtttacgcggtatcgatgttcaacccgactggtaatgacatgaccaagggtttgttgaccttggccaaaggtaaaccgattggcaaagaaggttactattggttgaagatccacggtgcgaactgcgcaggggtggataaggtaccgttcccggaacgtattaaattcatcgaggaaaaccacgaaaacattatggcgtgcgcaaagagcccgctggaaaacacgtggtgggcagagcaggacagtccattctgcttcttggcgttctgtttcgaatatgcaggtgtccagcaccacggcctgagctataactgcagcctgccgctggcctttgatggttcttgtagcggtattcaacactttagcgccatgctgcgcgatgaggttggtggcagagcagtgaatctgctgccaagcgaaaccgtgcaagatatctatggcattgtggctaagaaggttaatgaaatcctgcaagcagacgcgattaacggcacggacaacgaggttgtcaccgtgaccgatgaaaacaccggtgagatctcggagaaagtgaaactgggcaccaaagccttggctggccaatggctggcatacggcgttactcgctccgtgaccaagcgttcggtgatgacccttgcttacggcagcaaagagtttggtttccgccaacaggttctggaggatactatccaaccggccatcgactctggtaaaggcctgatgttcacgcagccgaatcaggcagcgggctatatggcgaagctgatttgggaatcggttagcgttaccgttgttgcagcggtggaggctatgaactggctgaaatctgcggcgaagctgttagctgcggaggtgaaggacaagaagacgggcgaaatcctgcgtaagcgctgcgcagtgcattgggttacgccggatggttttccggtatggcaggagtacaaaaagcctattcagacccgtctgaacctgatgtttctgggtcaatttcgtctgcagccgacgatcaacaccaataaggactccgagatcgacgcgcacaaacaggagtctggcatcgcacccaatttcgttcactcacaggacggttcccatctgcgtaagaccgtcgtgtgggcacacgagaagtatggcattgagtcgtttgcattgatccacgattcctttggtaccatcccggcggacgctgcgaacctgtttaaagcggttcgcgaaaccatggttgacacctatgaaagttgcgatgttctggcagacttttatgatcagttcgccgaccaactgcatgagtcccagctggataaaatgccggcgttaccggcgaagggcaacttaaatctccgcgacatcctggaatctgatttcgccttcgcgtaa

SEQ ID NO: 30 - DNA, 2652 bp, synthetic construct
  source 1..2652: mol_type = other DNA
atgaatacaattaacatagctaaaaatgatttcagcgatattgaactggctgcgatcccgtttaataccttggcggaccattatggtgagcgtctggcgcgtgagcaacttgctctggagcacgaatcctacgagatgggtgaagcgcgtttccggaagatgttcgagcgccagcttaaggctggcgaggtggcggataacgctgctgcgaagccgttgattacgaccctgctgccgaaaatgattgcgcgtattaacgattggttcgaggaagtgaaagcaaagcgtggtaaacgtccaaccgcattccagtttctgcaagagatcaagccggaggcggtggcatacattacgatcaaaaccactctcgcatgtctcaccagcgcggataatactacggtccaagcggtggccagcgcgattggccgcgcgattgaggacgaagcgcgttttggtcgcattcgtgacctggaagcgaaacattttaagaagaacgttgaagaacaattgaataaacgcgtgggccacgtttacaagaaagcgttcatgcaagtcgttgaagctgatatgctgagcaaaggcctgttaggtggtgaagcatggagcagctggcataaggaggactcaattcacgtcggcgtgcggtgcattgaaatgctgatcgaatcgaccggtatggttagcctgcatcgccaaaacgccggcgtggtgggtcaagatagcgaaacgattgaactggcgccagagtacgcggaagctatcgctaccagagccggcgcattggcggggatcagcccgatgttccagccgtgtgttgtaccaccgaagccgtggaccggtatcaccggtggaggttactgggcgaatggtagacgtccgttggcgttggttcgtacccatagcaaaaaggctctgatgcgttatgaagacgtttacatgccggaagtgtacaaagccatcaacatcgcgcagaacactgcgtggaaaatcaacaaaaaggtgttagctgtggcgaacgtaattacaaaatggaagcactgcccggttgaggacatcccggctattgaacgtgaagagctgccaatgaaaccagaggacattgacatgaatccggaggcgctgaccgcatggaaacgtgcggcagcagcggtctatcgtaaggataaagccagaaagagccgtcgtatctccctggaattcatgcttgagcaggcgaacaaattcgctaaccacaaagccatctggtttccgtataatatggattggcgtggtcgtgtttacgcggtatcgatgttcaacccgcagggttttgacatgaccaagggtttgttgaccttggccaaaggtaaaccgattggcaaagaaggttactattggttgaagatccacggtgcgaactgcgcaggggtggataaggtaccgttcccggaacgtattaaattcatcgaggaaaaccacgaaaacattatggcgtgcgcaaagagcccgctggaaaacacgtggtgggcagagcaggacagtccattctgcttcttggcgttctgtttcgaatatgcaggtgtccagcaccacggcctgagctataactgcagcctgccgctggcctttgatggttcttgtagcggtattcaacactttagcgccatgctgcgcgatgaggttggtggcagagcagtgaatctgctgccaagcgaaaccgtgcaagatatctatggcattgtggctaagaaggttaatgaaatcctgcaagcagacgcgattaacggcacggacaacgaggttgtcaccgtgaccgatgaaaacaccggtgagatctcggagaaagtgaaactgggcaccaaagccttggctggccaatggctggcatacggcgttactcgctccgtgaccaagcgttcggtgatgacccttgcttacggcagcaaagagtttggtttccgccaacaggttctggaggatactatccaaccggccatcgactctggtaaaggcctgatgttcacgcagccgaatcaggcagcgggctatatggcgaagctgatttgggaatcggttagcgttaccgttgttgcagcggtggaggctatgaactggctgaaatctgcggcgaagctgttagctgcggaggtgaaggacaagaagacgggcgaaatcctgcgtaagcgctgcgcagtgcattgggttacgccggatggttttccggtatggcaggagtacaaaaagcctattcagacccgtctgaacctgatgtttctgggtcaatttcgtctgcagccgacgatcaacaccaataaggactccgagatcgacgcgcacaaacaggagtctggcatcgcacccaatttcgttcactcacaggacggttcccatctgcgtaagaccgtcgtgtgggcacacgagaagtatggcattgagtcgtttgcattgatccacgattcctttggtaccatcccggcggacgctgcgaacctgtttaaagcggttcgcgaaaccatggttgacacctatgaaagttgcgatgttctggcagacttttatgatcagttcgccgaccaactgcatgagtcccagctggataaaatgccggcgttaccggcgaagggcaacttaaatctccgcgacatcctggaatctgatttcgccttcgcgtaa

SEQ ID NO: 31 - DNA, 2652 bp, synthetic construct
  source 1..2652: mol_type = other DNA
atgaatacaattaacatagctaaaaatgatttcagcgatattgaactggctgcgatcccgtttaataccttggcggaccattatggtgagcgtctggcgcgtgagcaacttgctctggagcacgaatcctacgagatgggtgaagcgcgtttccggaagatgttcgagcgccagcttaaggctggcgaggtggcggataacgctgctgcgaagccgttgattacgaccctgctgccgaaaatgattgcgcgtattaacgattggttcgaggaagtgaaagcaaagcgtggtaaacgtccaaccgcattccagtttctgcaagagatcaagccggaggcggtggcatacattacgatcaaaaccactctcgcatgtctcaccagcgcggataatactacggtccaagcggtggccagcgcgattggccgcgcgattgaggacgaagcgcgttttggtcgcattcgtgacctggaagcgaaacattttaagaagaacgttgaagaacaattgaataaacgcgtgggccacgtttacaagaaagcgttcatgcaagtcgttgaagctgatatgctgagcaaaggcctgttaggtggtgaagcatggagcagctggcataaggaggactcaattcacgtcggcgtgcggtgcattgaaatgctgatcgaatcgaccggtatggttagcctgcatcgccaaaacgccggcgtggtgggtcaagatagcgaaacgattgaactggcgccagagtacgcggaagctatcgctaccagagccggcgcattggcggggatcagcccgatgttccagccgtgtgttgtaccaccgaagccgtggaccggtatcaccggtggaggttactgggcgaatggtagacgtccgttggcgttggttcgtacccatagcaaaaaggctctgatgcgttatgaagacgtttacatgccggaagtgtacaaagccatcaacatcgcgcagaacactgcgtggaaaatcaacaaaaaggtgttagctgtggcgaacgtaattacaaaatggaagcactgcccggttgaggacatcccggctattgaacgtgaagagctgccaatgaaaccagaggacattgacatgaatccggaggcgctgaccgcatggaaacgtgcggcagcagcggtctatcgtaaggataaagccagaaagagccgtcgtatctccctggaattcatgcttgagcaggcgaacaaattcgctaaccacaaagccatctggtttccgtataatatggattggcgtggtcgtgtttacgcggtatcgatgttcaacccgcagggtactgacatgaccaagggtttgttgaccttggccaaaggtaaaccgattggcaaagaaggttactattggttgaagatccacggtgcgaactgcgcaggggtggataaggtaccgttcccggaacgtattaaattcatcgaggaaaaccacgaaaacattatggcgtgcgcaaagagcccgctggaaaacacgtggtgggcagagcaggacagtccattctgcttcttggcgttctgtttcgaatatgcaggtgtccagcaccacggcctgagctataactgcagcctgccgctggcctttgatggttcttgtagcggtattcaacactttagcgccatgctgcgcgatgaggttggtggcagagcagtgaatctgctgccaagcgaaaccgtgcaagatatctatggcattgtggctaagaaggttaatgaaatcctgcaagcagacgcgattaacggcacggacaacgaggttgtcaccgtgaccgatgaaaacaccggtgagatctcggagaaagtgaaactgggcaccaaagccttggctggccaatggctggcatacggcgttactcgctccgtgaccaagcgttcggtgatgacccttgcttacggcagcaaagagtttggtttccgccaacaggttctggaggatactatccaaccggccatcgactctggtaaaggcctgatgttcacgcagccgaatcaggcagcgggctatatggcgaagctgatttgggaatcggttagcgttaccgttgttgcagcggtggaggctatgaactggctgaaatctgcggcgaagctgttagctgcggaggtgaaggacaagaagacgggcgaaatcctgcgtaagcgctgcgcagtgcattgggttacgccggatggttttccggtatggcaggagtacaaaaagcctattcagacccgtctgaacctgatgtttctgggtcaatttcgtctgcagccgacgatcaacaccaataaggactccgagatcgacgcgcacaaacaggagtctggcatcgcacccaatttcgttcactcacaggacggttcccatctgcgtaagaccgtcgtgtgggcacacgagaagtatggcattgagtcgtttgcattgatccacgattcctttggtaccatcccggcggacgctgcgaacctgtttaaagcggttcgcgaaaccatggttgacacctatgaaagttgcgatgttctggcagacttttatgatcagttcgccgaccaactgcatgagtcccagctggataaaatgccggcgttaccggcgaagggcaacttaaatctccgcgacatcctggaatctgatttcgccttcgcgtaa

SEQ ID NO: 32 - DNA, 2652 bp, synthetic construct
  source 1..2652: mol_type = other DNA
atgaatacaattaacatagctaaaaatgatttcagcgatattgaactggctgcgatcccgtttaataccttggcggaccattatggtgagcgtctggcgcgtgagcaacttgctctggagcacgaatcctacgagatgggtgaagcgcgtttccggaagatgttcgagcgccagcttaaggctggcgaggtggcggataacgctgctgcgaagccgttgattacgaccctgctgccgaaaatgattgcgcgtattaacgattggttcgaggaagtgaaagcaaagcgtggtaaacgtccaaccgcattccagtttctgcaagagatcaagccggaggcggtggcatacattacgatcaaaaccactctcgcatgtctcaccagcgcggataatactacggtccaagcggtggccagcgcgattggccgcgcgattgaggacgaagcgcgttttggtcgcattcgtgacctggaagcgaaacattttaagaagaacgttgaagaacaattgaataaacgcgtgggccacgtttacaagaaagcgttcatgcaagtcgttgaagctgatatgctgagcaaaggcctgttaggtggtgaagcatggagcagctggcataaggaggactcaattcacgtcggcgtgcggtgcattgaaatgctgatcgaatcgaccggtatggttagcctgcatcgccaaaacgccggcgtggtgggtcaagatagcgaaacgattgaactggcgccagagtacgcggaagctatcgctaccagagccggcgcattggcggggatcagcccgatgttccagccgtgtgttgtaccaccgaagccgtggaccggtatcaccggtggaggttactgggcgaatggtagacgtccgttggcgttggttcgtacccatagcaaaaaggctctgatgcgttatgaagacgtttacatgccggaagtgtacaaagccatcaacatcgcgcagaacactgcgtggaaaatcaacaaaaaggtgttagctgtggcgaacgtaattacaaaatggaagcactgcccggttgaggacatcccggctattgaacgtgaagagctgccaatgaaaccagaggacattgacatgaatccggaggcgctgaccgcatggaaacgtgcggcagcagcggtctatcgtaaggataaagccagaaagagccgtcgtatctccctggaattcatgcttgagcaggcgaacaaattcgctaaccacaaagccatctggtttccgtataatatggattggcgtggtcgtgtttacgcggtatcgatgttcaacccgcagggtaatactatgaccaagggtttgttgaccttggccaaaggtaaaccgattggcaaagaaggttactattggttgaagatccacggtgcgaactgcgcaggggtggataaggtaccgttcccggaacgtattaaattcatcgaggaaaaccacgaaaacattatggcgtgcgcaaagagcccgctggaaaacacgtggtgggcagagcaggacagtccattctgcttcttggcgttctgtttcgaatatgcaggtgtccagcaccacggcctgagctataactgcagcctgccgctggcctttgatggttcttgtagcggtattcaacactttagcgccatgctgcgcgatgaggttggtggcagagcagtgaatctgctgccaagcgaaaccgtgcaagatatctatggcattgtggctaagaaggttaatgaaatcctgcaagcagacgcgattaacggcacggacaacgaggttgtcaccgtgaccgatgaaaacaccggtgagatctcggagaaagtgaaactgggcaccaaagccttggctggccaatggctggcatacggcgttactcgctccgtgaccaagcgttcggtgatgacccttgcttacggcagcaaagagtttggtttccgccaacaggttctggaggatactatccaaccggccatcgactctggtaaaggcctgatgttcacgcagccgaatcaggcagcgggctatatggcgaagctgatttgggaatcggttagcgttaccgttgttgcagcggtggaggctatgaactggctgaaatctgcggcgaagctgttagctgcggaggtgaaggacaagaagacgggcgaaatcctgcgtaagcgctgcgcagtgcattgggttacgccggatggttttccggtatggcaggagtacaaaaagcctattcagacccgtctgaacctgatgtttctgggtcaatttcgtctgcagccgacgatcaacaccaataaggactccgagatcgacgcgcacaaacaggagtctggcatcgcacccaatttcgttcactcacaggacggttcccatctgcgtaagaccgtcgtgtgggcacacgagaagtatggcattgagtcgtttgcattgatccacgattcctttggtaccatcccggcggacgctgcgaacctgtttaaagcggttcgcgaaaccatggttgacacctatgaaagttgcgatgttctggcagacttttatgatcagttcgccgaccaactgcatgagtcccagctggataaaatgccggcgttaccggcgaagggcaacttaaatctccgcgacatcctggaatctgatttcgccttcgcgtaa

SEQ ID NO: 33 - DNA, 2652 bp, synthetic construct
  source 1..2652: mol_type = other DNA
atgaatacaattaacatagctaaaaatgatttcagcgatattgaactggctgcgatcccgtttaataccttggcggaccattatggtgagcgtctggcgcgtgagcaacttgctctggagcacgaatcctacgagatgggtgaagcgcgtttccggaagatgttcgagcgccagcttaaggctggcgaggtggcggataacgctgctgcgaagccgttgattacgaccctgctgccgaaaatgattgcgcgtattaacgattggttcgaggaagtgaaagcaaagcgtggtaaacgtccaaccgcattccagtttctgcaagagatcaagccggaggcggtggcatacattacgatcaaaaccactctcgcatgtctcaccagcgcggataatactacggtccaagcggtggccagcgcgattggccgcgcgattgaggacgaagcgcgttttggtcgcattcgtgacctggaagcgaaacattttaagaagaacgttgaagaacaattgaataaacgcgtgggccacgtttacaagaaagcgttcatgcaagtcgttgaagctgatatgctgagcaaaggcctgttaggtggtgaagcatggagcagctggcataaggaggactcaattcacgtcggcgtgcggtgcattgaaatgctgatcgaatcgaccggtatggttagcctgcatcgccaaaacgccggcgtggtgggtcaagatagcgaaacgattgaactggcgccagagtacgcggaagctatcgctaccagagccggcgcattggcggggatcagcccgatgttccagccgtgtgttgtaccaccgaagccgtggaccggtatcaccggtggaggttactgggcgaatggtagacgtccgttggcgttggttcgtacccatagcaaaaaggctctgatgcgttatgaagacgtttacatgccggaagtgtacaaagccatcaacatcgcgcagaacactgcgtggaaaatcaacaaaaaggtgttagctgtggcgaacgtaattacaaaatggaagcactgcccggttgaggacatcccggctattgaacgtgaagagctgccaatgaaaccagaggacattgacatgaatccggaggcgctgaccgcatggaaacgtgcggcagcagcggtctatcgtaaggataaagccagaaagagccgtcgtatctccctggaattcatgcttgagcaggcgaacaaattcgctaaccacaaagccatctggtttccgtataatatggattggcgtggtcgtgtttacgcggtatcgatgttcaacccgcagggtaatcttatgaccaagggtttgttgaccttggccaaaggtaaaccgattggcaaagaaggttactattggttgaagatccacggtgcgaactgcgcaggggtggataaggtaccgttcccggaacgtattaaattcatcgaggaaaaccacgaaaacattatggcgtgcgcaaagagcccgctggaaaacacgtggtgggcagagcaggacagtccattctgcttcttggcgttctgtttcgaatatgcaggtgtccagcaccacggcctgagctataactgcagcctgccgctggcctttgatggttcttgtagcggtattcaacactttagcgccatgctgcgcgatgaggttggtggcagagcagtgaatctgctgccaagcgaaaccgtgcaagatatctatggcattgtggctaagaaggttaatgaaatcctgcaagcagacgcgattaacggcacggacaacgaggttgtcaccgtgaccgatgaaaacaccggtgagatctcggagaaagtgaaactgggcaccaaagccttggctggccaatggctggcatacggcgttactcgctccgtgaccaagcgttcggtgatgacccttgcttacggcagcaaagagtttggtttccgccaacaggttctggaggatactatccaaccggccatcgactctggtaaaggcctgatgttcacgcagccgaatcaggcagcgggctatatggcgaagctgatttgggaatcggttagcgttaccgttgttgcagcggtggaggctatgaactggctgaaatctgcggcgaagctgttagctgcggaggtgaaggacaagaagacgggcgaaatcctgcgtaagcgctgcgcagtgcattgggttacgccggatggttttccggtatggcaggagtacaaaaagcctattcagacccgtctgaacctgatgtttctgggtcaatttcgtctgcagccgacgatcaacaccaataaggactccgagatcgacgcgcacaaacaggagtctggcatcgcacccaatttcgttcactcacaggacggttcccatctgcgtaagaccgtcgtgtgggcacacgagaagtatggcattgagtcgtttgcattgatccacgattcctttggtaccatcccggcggacgctgcgaacctgtttaaagcggttcgcgaaaccatggttgacacctatgaaagttgcgatgttctggcagacttttatgatcagttcgccgaccaactgcatgagtcccagctggataaaatgccggcgttaccggcgaagggcaacttaaatctccgcgacatcctggaatctgatttcgccttcgcgtaa

SEQ ID NO: 34 - DNA, 2652 bp, synthetic construct
  source 1..2652: mol_type = other DNA
atgaatacaattaacatagctaaaaatgatttcagcgatattgaactggctgcgatcccgtttaataccttggcggaccattatggtgagcgtctggcgcgtgagcaacttgctctggagcacgaatcctacgagatgggtgaagcgcgtttccggaagatgttcgagcgccagcttaaggctggcgaggtggcggataacgctgctgcgaagccgttgattacgaccctgctgccgaaaatgattgcgcgtattaacgattggttcgaggaagtgaaagcaaagcgtggtaaacgtccaaccgcattccagtttctgcaagagatcaagccggaggcggtggcatacattacgatcaaaaccactctcgcatgtctcaccagcgcggataatactacggtccaagcggtggccagcgcgattggccgcgcgattgaggacgaagcgcgttttggtcgcattcgtgacctggaagcgaaacattttaagaagaacgttgaagaacaattgaataaacgcgtgggccacgtttacaagaaagcgttcatgcaagtcgttgaagctgatatgctgagcaaaggcctgttaggtggtgaagcatggagcagctggcataaggaggactcaattcacgtcggcgtgcggtgcattgaaatgctgatcgaatcgaccggtatggttagcctgcatcgccaaaacgccggcgtggtgggtcaagatagcgaaacgattgaactggcgccagagtacgcggaagctatcgctaccagagccggcgcattggcggggatcagcccgatgttccagccgtgtgttgtaccaccgaagccgtggaccggtatcaccggtggaggttactgggcgaatggtagacgtccgttggcgttggttcgtacccatagcaaaaaggctctgatgcgttatgaagacgtttacatgccggaagtgtacaaagccatcaacatcgcgcagaacactgcgtggaaaatcaacaaaaaggtgttagctgtggcgaacgtaattacaaaatggaagcactgcccggttgaggacatcccggctattgaacgtgaagagctgccaatgaaaccagaggacattgacatgaatccggaggcgctgaccgcatggaaacgtgcggcagcagcggtctatcgtaaggataaagccagaaagagccgtcgtatctccctggaattcatgcttgagcaggcgaacaaattcgctaaccacaaagccatctggtttccgtataatatggattggcgtggtcgtgtttacgcggtatcgatgttcaacccgcagggtaatattatgaccaagggtttgttgaccttggccaaaggtaaaccgattggcaaagaaggttactattggttgaagatccacggtgcgaactgcgcaggggtggataaggtaccgttcccggaacgtattaaattcatcgaggaaaaccacgaaaacattatggcgtgcgcaaagagcccgctggaaaacacgtggtgggcagagcaggacagtccattctgcttcttggcgttctgtttcgaatatgcaggtgtccagcaccacggcctgagctataactgcagcctgccgctggcctttgatggttcttgtagcggtattcaacactttagcgccatgctgcgcgatgaggttggtggcagagcagtgaatctgctgccaagcgaaaccgtgcaagatatctatggcattgtggctaagaaggttaatgaaatcctgcaagcagacgcgattaacggcacggacaacgaggttgtcaccgtgaccgatgaaaacaccggtgagatctcggagaaagtgaaactgggcaccaaagccttggctggccaatggctggcatacggcgttactcgctccgtgaccaagcgttcggtgatgacccttgcttacggcagcaaagagtttggtttccgccaacaggttctggaggatactatccaaccggccatcgactctggtaaaggcctgatgttcacgcagccgaatcaggcagcgggctatatggcgaagctgatttgggaatcggttagcgttaccgttgttgcagcggtggaggctatgaactggctgaaatctgcggcgaagctgttagctgcggaggtgaaggacaagaagacgggcgaaatcctgcgtaagcgctgcgcagtgcattgggttacgccggatggttttccggtatggcaggagtacaaaaagcctattcagacccgtctgaacctgatgtttctgggtcaatttcgtctgcagccgacgatcaacaccaataaggactccgagatcgacgcgcacaaacaggagtctggcatcgcacccaatttcgttcactcacaggacggttcccatctgcgtaagaccgtcgtgtgggcacacgagaagtatggcattgagtcgtttgcattgatccacgattcctttggtaccatcccggcggacgctgcgaacctgtttaaagcggttcgcgaaaccatggttgacacctatgaaagttgcgatgttctggcagacttttatgatcagttcgccgaccaactgcatgagtcccagctggataaaatgccggcgttaccggcgaagggcaacttaaatctccgcgacatcctggaatctgatttcgccttcgcgtaa

SEQ ID NO: 35 - DNA, 2652 bp, synthetic construct
  source 1..2652: mol_type = other DNA
atgaatacaattaacatagctaaaaatgatttcagcgatattgaactggctgcgatcccgtttaataccttggcggaccattatggtgagcgtctggcgcgtgagcaacttgctctggagcacgaatcctacgagatgggtgaagcgcgtttccggaagatgttcgagcgccagcttaaggctggcgaggtggcggataacgctgctgcgaagccgttgattacgaccctgctgccgaaaatgattgcgcgtattaacgattggttcgaggaagtgaaagcaaagcgtggtaaacgtccaaccgcattccagtttctgcaagagatcaagccggaggcggtggcatacattacgatcaaaaccactctcgcatgtctcaccagcgcggataatactacggtccaagcggtggccagcgcgattggccgcgcgattgaggacgaagcgcgttttggtcgcattcgtgacctggaagcgaaacattttaagaagaacgttgaagaacaattgaataaacgcgtgggccacgtttacaagaaagcgttcatgcaagtcgttgaagctgatatgctgagcaaaggcctgttaggtggtgaagcatggagcagctggcataaggaggactcaattcacgtcggcgtgcggtgcattgaaatgctgatcgaatcgaccggtatggttagcctgcatcgccaaaacgccggcgtggtgggtcaagatagcgaaacgattgaactggcgccagagtacgcggaagctatcgctaccagagccggcgcattggcggggatcagcccgatgttccagccgtgtgttgtaccaccgaagccgtggaccggtatcaccggtggaggttactgggcgaatggtagacgtccgttggcgttggttcgtacccatagcaaaaaggctctgatgcgttatgaagacgtttacatgccggaagtgtacaaagccatcaacatcgcgcagaacactgcgtggaaaatcaacaaaaaggtgttagctgtggcgaacgtaattacaaaatggaagcactgcccggttgaggacatcccggctattgaacgtgaagagctgccaatgaaaccagaggacattgacatgaatccggaggcgctgaccgcatggaaacgtgcggcagcagcggtctatcgtaaggataaagccagaaagagccgtcgtatctccctggaattcatgcttgagcaggcgaacaaattcgctaaccacaaagccatctggtttccgtataatatggattggcgtggtcgtgtttacgcggtatcgatgttcaacccgcagggtaatcctatgaccaagggtttgttgaccttggccaaaggtaaaccgattggcaaagaaggttactattggttgaagatccacggtgcgaactgcgcaggggtggataaggtaccgttcccggaacgtattaaattcatcgaggaaaaccacgaaaacattatggcgtgcgcaaagagcccgctggaaaacacgtggtgggcagagcaggacagtccattctgcttcttggcgttctgtttcgaatatgcaggtgtccagcaccacggcctgagctataactgcagcctgccgctggcctttgatggttcttgtagcggtattcaacactttagcgccatgctgcgcgatgaggttggtggcagagcagtgaatctgctgccaagcgaaaccgtgcaagatatctatggcattgtggctaagaaggttaatgaaatcctgcaagcagacgcgattaacggcacggacaacgaggttgtcaccgtgaccgatgaaaacaccggtgagatctcggagaaagtgaaactgggcaccaaagccttggctggccaatggctggcatacggcgttactcgctccgtgaccaagcgttcggtgatgacccttgcttacggcagcaaagagtttggtttccgccaacaggttctggaggatactatccaaccggccatcgactctggtaaaggcctgatgttcacgcagccgaatcaggcagcgggctatatggcgaagctgatttgggaatcggttagcgttaccgttgttgcagcggtggaggctatgaactggctgaaatctgcggcgaagctgttagctgcggaggtgaaggacaagaagacgggcgaaatcctgcgtaagcgctgcgcagtgcattgggttacgccggatggttttccggtatggcaggagtacaaaaagcctattcagacccgtctgaacctgatgtttctgggtcaatttcgtctgcagccgacgatcaacaccaataaggactccgagatcgacgcgcacaaacaggagtctggcatcgcacccaatttcgttcactcacaggacggttcccatctgcgtaagaccgtcgtgtgggcacacgagaagtatggcattgagtcgtttgcattgatccacgattcctttggtaccatcccggcggacgctgcgaacctgtttaaagcggttcgcgaaaccatggttgacacctatgaaagttgcgatgttctggcagacttttatgatcagttcgccgaccaactgcatgagtcccagctggataaaatgccggcgttaccggcgaagggcaacttaaatctccgcgacatcctggaatctgatttcgccttcgcgtaa

SEQ ID NO: 36 - DNA, 2652 bp, synthetic construct
  source 1..2652: mol_type = other DNA
atgaatacaattaacatagctaaaaatgatttcagcgatattgaactggctgcgatcccgtttaataccttggcggaccattatggtgagcgtctggcgcgtgagcaacttgctctggagcacgaatcctacgagatgggtgaagcgcgtttccggaagatgttcgagcgccagcttaaggctggcgaggtggcggataacgctgctgcgaagccgttgattacgaccctgctgccgaaaatgattgcgcgtattaacgattggttcgaggaagtgaaagcaaagcgtggtaaacgtccaaccgcattccagtttctgcaagagatcaagccggaggcggtggcatacattacgatcaaaaccactctcgcatgtctcaccagcgcggataatactacggtccaagcggtggccagcgcgattggccgcgcgattgaggacgaagcgcgttttggtcgcattcgtgacctggaagcgaaacattttaagaagaacgttgaagaacaattgaataaacgcgtgggccacgtttacaagaaagcgttcatgcaagtcgttgaagctgatatgctgagcaaaggcctgttaggtggtgaagcatggagcagctggcataaggaggactcaattcacgtcggcgtgcggtgcattgaaatgctgatcgaatcgaccggtatggttagcctgcatcgccaaaacgccggcgtggtgggtcaagatagcgaaacgattgaactggcgccagagtacgcggaagctatcgctaccagagccggcgcattggcggggatcagcccgatgttccagccgtgtgttgtaccaccgaagccgtggaccggtatcaccggtggaggttactgggcgaatggtagacgtccgttggcgttggttcgtacccatagcaaaaaggctctgatgcgttatgaagacgtttacatgccggaagtgtacaaagccatcaacatcgcgcagaacactgcgtggaaaatcaacaaaaaggtgttagctgtggcgaacgtaattacaaaatggaagcactgcccggttgaggacatcccggctattgaacgtgaagagctgccaatgaaaccagaggacattgacatgaatccggaggcgctgaccgcatggaaacgtgcggcagcagcggtctatcgtaaggataaagccagaaagagccgtcgtatctccctggaattcatgcttgagcaggcgaacaaattcgctaaccacaaagccatctggtttccgtataatatggattggcgtggtcgtgtttacgcggtatcgatgttcaacccgcagggtaatgttatgaccaagggtttgttgaccttggccaaaggtaaaccgattggcaaagaaggttactattggttgaagatccacggtgcgaactgcgcaggggtggataaggtaccgttcccggaacgtattaaattcatcgaggaaaaccacgaaaacattatggcgtgcgcaaagagcccgctggaaaacacgtggtgggcagagcaggacagtccattctgcttcttggcgttctgtttcgaatatgcaggtgtccagcaccacggcctgagctataactgcagcctgccgctggcctttgatggttcttgtagcggtattcaacactttagcgccatgctgcgcgatgaggttggtggcagagcagtgaatctgctgccaagcgaaaccgtgcaagatatctatggcattgtggctaagaaggttaatgaaatcctgcaagcagacgcgattaacggcacggacaacgaggttgtcaccgtgaccgatgaaaacaccggtgagatctcggagaaagtgaaactgggcaccaaagccttggctggccaatggctggcatacggcgttactcgctccgtgaccaagcgttcggtgatgacccttgcttacggcagcaaagagtttggtttccgccaacaggttctggaggatactatccaaccggccatcgactctggtaaaggcctgatgttcacgcagccgaatcaggcagcgggctatatggcgaagctgatttgggaatcggttagcgttaccgttgttgcagcggtggaggctatgaactggctgaaatctgcggcgaagctgttagctgcggaggtgaaggacaagaagacgggcgaaatcctgcgtaagcgctgcgcagtgcattgggttacgccggatggttttccggtatggcaggagtacaaaaagcctattcagacccgtctgaacctgatgtttctgggtcaatttcgtctgcagccgacgatcaacaccaataaggactccgagatcgacgcgcacaaacaggagtctggcatcgcacccaatttcgttcactcacaggacggttcccatctgcgtaagaccgtcgtgtgggcacacgagaagtatggcattgagtcgtttgcattgatccacgattcctttggtaccatcccggcggacgctgcgaacctgtttaaagcggttcgcgaaaccatggttgacacctatgaaagttgcgatgttctggcagacttttatgatcagttcgccgaccaactgcatgagtcccagctggataaaatgccggcgttaccggcgaagggcaacttaaatctccgcgacatcctggaatctgatttcgccttcgcgtaa

SEQ ID NO: 37 - DNA, 2652 bp, synthetic construct
  source 1..2652: mol_type = other DNA
atgaatacaattaacatagctaaaaatgatttcagcgatattgaactggctgcgatcccgtttaataccttggcggaccattatggtgagcgtctggcggctgagcaacttgctctggagcacgaatcctacgagatgggtgaagcgcgtttccggaagatgttcgagcgccagcttaaggctggcgaggtggcggataacgctgctgcgaagccgttgattacgaccctgctgccgaaaatgattgcgcgtattaacgattggttcgaggaagtgaaagcaaagcgtggtaaacgtccaaccgcattccagtttctgcaagagatcaagccggaggcggtggcatacattacgatcaaaaccactctcgcatgtctcaccagcgcggataatactacggtccaagcggtggccagcgcgattggccgcgcgattgaggacgaagcgcgttttggtcgcattcgtgacctggaagcgaaacattttaagaagaacgttgaagaacaattgaataaacgcgtgggccacgtttacaagaaagcgttcatgcaagtcgttgaagctgatatgctgagcaaaggcctgttaggtggtgaagcatggagcagctggcataaggaggactcaattcacgtcggcgtgcggtgcattgaaatgctgatcgaatcgaccggtatggttagcctgcatcgccaaaacgccggcgtggtgggtcaagatagcgaaacgattgaactggcgccagagtacgcggaagctatcgctaccagagccggcgcattggcggggatcagcccgatgttccagccgtgtgttgtaccaccgaagccgtggaccggtatcaccggtggaggttactgggcgaatggtagacgtccgttggcgttggttcgtacccatagcaaaaaggctctgatgcgttatgaagacgtttacatgccggaagtgtacaaagccatcaacatcgcgcagaacactgcgtggaaaatcaacaaaaaggtgttagctgtggcgaacgtaattacaaaatggaagcactgcccggttgaggacatcccggctattgaacgtgaagagctgccaatgaaaccagaggacattgacatgaatccggaggcgctgaccgcatggaaacgtgcggcagcagcggtctatgctaaggataaagccagaaagagccgtcgtatctccctggaattcatgcttgagcaggcgaacaaattcgctaaccacaaagccatctggtttccgtataatatggattggcgtggtcgtgtttacgcggtatcgatgttcaacccgcagggtaatgacatgaccaagggtttgttgaccttggccaaaggtaaaccgattggcaaagaaggttactattggttgaagatccacggtgcgaactgcgcaggggtggataaggtaccgttcccggaacgtattaaattcatcgaggaaaaccacgaaaacattatggcgtgcgcaaagagcccgctggaaaacacgtggtgggcagagcaggacagtccattctgcttcttggcgttctgtttcgaatatgcaggtgtccagcaccacggcctgagctataactgcagcctgccgctggcctttgatggttcttgtagcggtattcaacactttagcgccatgctgcgcgatgaggttggtggcagagcagtgaatctgctgccaagcgaaaccgtgcaagatatctatggcattgtggctaagaaggttaatgaaatcctgcaagcagacgcgattaacggcacggacaacgaggttgtcaccgtgaccgatgaaaacaccggtgagatctcggagaaagtgaaactgggcaccaaagccttggctggccaatggctggcatacggcgttactcgctccgtgaccaagcgttcggtgatgacccttgcttacggcagcaaagagtttggtttccgccaacaggttctggaggatactatccaaccggccatcgactctggtaaaggcctgatgttcacgcagccgaatcaggcagcgggctatatggcgaagctgatttgggaatcggttagcgttaccgttgttgcagcggtggaggctatgaactggctgaaatctgcggcgaagctgttagctgcggaggtgaaggacaagaagacgggcgaaatcctgcgtaagcgctgcgcagtgcattgggttacgccggatggttttccggtatggcaggagtacaaaaagcctattcagacccgtctgaacctgatgtttctgggtcaatttcgtctgcagccgacgatcaacaccaataaggactccgagatcgacgcgcacaaacaggagtctggcatcgcacccaatttcgttcactcacaggacggttcccatctgcgtaagaccgtcgtgtgggcacacgagaagtatggcattgagtcgtttgcattgatccacgattcctttggtaccatcccggcggacgctgcgaacctgtttaaagcggttcgcgaaaccatggttgacacctatgaaagttgcgatgttctggcagacttttatgatcagttcgccgaccaactgcatgagtcccagctggataaaatgccggcgttaccggcgaagggcaacttaaatctccgcgacatcctggaatctgatttcgccttcgcgtaa

SEQ ID NO: 38 - DNA, 2652 bp, synthetic construct
  source 1..2652: mol_type = other DNA
atgaatacaattaacatagctaaaaatgatttcagcgatattgaactggctgcgatcccgtttaataccttggcggaccattatggtgagcgtctggcggctgagcaacttgctctggagcacgaatcctacgagatgggtgaagcgcgtttccggaagatgttcgagcgccagcttaaggctggcgaggtggcggataacgctgctgcgaagccgttgattacgaccctgctgccgaaaatgattgcgcgtattaacgattggttcgaggaagtgaaagcaaagcgtggtaaacgtccaaccgcattccagtttctgcaagagatcaagccggaggcggtggcatacattacgatcaaaaccactctcgcatgtctcaccagcgcggataatactacggtccaagcggtggccagcgcgattggccgcgcgattgaggacgaagcgcgttttggtcgcattcgtgacctggaagcgaaacattttaagaagaacgttgaagaacaattgaataaacgcgtgggccacgtttacaagaaagcgttcatgcaagtcgttgaagctgatatgctgagcaaaggcctgttaggtggtgaagcatggagcagctggcataaggaggactcaattcacgtcggcgtgcggtgcattgaaatgctgatcgaatcgaccggtatggttagcctgcatcgccaaaacgccggcgtggtgggtcaagatagcgaaacgattgaactggcgccagagtacgcggaagctatcgctaccagagccggcgcattggcggggatcagcccgatgttccagccgtgtgttgtaccaccgaagccgtggaccggtatcaccggtggaggttactgggcgaatggtagacgtccgttggcgttggttcgtacccatagcaaaaaggctctgatgcgttatgaagacgtttacatgccggaagtgtacaaagccatcaacatcgcgcagaacactgcgtggaaaatcaacaaaaaggtgttagctgtggcgaacgtaattacaaaatggaagcactgcccggttgaggacatcccggctattgaacgtgaagagctgccaatgaaaccagaggacattgacatgaatccggaggcgctgaccgcatggaaacgtgcggcagcagcggtctatatgaaggataaagccagaaagagccgtcgtatctccctggaattcatgcttgagcaggcgaacaaattcgctaaccacaaagccatctggtttccgtataatatggattggcgtggtcgtgtttacgcggtatcgatgttcaacccgcagggtaatgacatgaccaagggtttgttgaccttggccaaaggtaaaccgattggcaaagaaggttactattggttgaagatccacggtgcgaactgcgcaggggtggataaggtaccgttcccggaacgtattaaattcatcgaggaaaaccacgaaaacattatggcgtgcgcaaagagcccgctggaaaacacgtggtgggcagagcaggacagtccattctgcttcttggcgttctgtttcgaatatgcaggtgtccagcaccacggcctgagctataactgcagcctgccgctggcctttgatggttcttgtagcggtattcaacactttagcgccatgctgcgcgatgaggttggtggcagagcagtgaatctgctgccaagcgaaaccgtgcaagatatctatggcattgtggctaagaaggttaatgaaatcctgcaagcagacgcgattaacggcacggacaacgaggttgtcaccgtgaccgatgaaaacaccggtgagatctcggagaaagtgaaactgggcaccaaagccttggctggccaatggctggcatacggcgttactcgctccgtgaccaagcgttcggtgatgacccttgcttacggcagcaaagagtttggtttccgccaacaggttctggaggatactatccaaccggccatcgactctggtaaaggcctgatgttcacgcagccgaatcaggcagcgggctatatggcgaagctgatttgggaatcggttagcgttaccgttgttgcagcggtggaggctatgaactggctgaaatctgcggcgaagctgttagctgcggaggtgaaggacaagaagacgggcgaaatcctgcgtaagcgctgcgcagtgcattgggttacgccggatggttttccggtatggcaggagtacaaaaagcctattcagacccgtctgaacctgatgtttctgggtcaatttcgtctgcagccgacgatcaacaccaataaggactccgagatcgacgcgcacaaacaggagtctggcatcgcacccaatttcgttcactcacaggacggttcccatctgcgtaagaccgtcgtgtgggcacacgagaagtatggcattgagtcgtttgcattgatccacgattcctttggtaccatcccggcggacgctgcgaacctgtttaaagcggttcgcgaaaccatggttgacacctatgaaagttgcgatgttctggcagacttttatgatcagttcgccgaccaactgcatgagtcccagctggataaaatgccggcgttaccggcgaagggcaacttaaatctccgcgacatcctggaatctgatttcgccttcgcgtaa

SEQ ID NO: 39 - DNA, 2652 bp, synthetic construct
  source 1..2652: mol_type = other DNA
atgaatacaattaacatagctaaaaatgatttcagcgatattgaactggctgcgatcccgtttaataccttggcggaccattatggtgagcgtctggcgcgtgagcaacttgctctggagcacgaatcctacgagatgggtgaagcgcgtttccggaagatgttcgagcgccagcttaaggctggcgaggtggcggataacgctgctgcgaagccgttgattacgaccctgctgccgaaaatgattgcgcgtattaacgattggttcgaggaagtgaaagcaaagcgtggtaaacgtccaaccgcattccagtttctgcaagagatcaagccggaggcggtggcatacattacgatcaaaaccactctcgcatgtctcaccagcgcggataatactacggtccaagcggtggccagcgcgattggccgcgcgattgaggacgaagcgcgttttggtcgcattcgtgacctggaagcgaaacattttaagaagaacgttgaagaacaattgaataaacgcgtgggccacgttcataagaaagcgttcatgcaagtcgttgaagctgatatgctgagcaaaggcctgttaggtggtgaagcatggagcagctggcataaggaggactcaattcacgtcggcgtgcggtgcattgaaatgctgatcgaatcgaccggtatggttagcctgcatcgccaaaacgccggcgtggtgggtcaagatagcgaaacgattgaactggcgccagagtacgcggaagctatcgctaccagagccggcgcattggcggggatcagcccgatgttccagccgtgtgttgtaccaccgaagccgtggaccggtatcaccggtggaggttactgggcgaatggtagacgtccgttggcgttggttcgtacccatagcaaaaaggctctgatgcgttatgaagacgtttacatgccggaagtgtacaaagccatcaacatcgcgcagaacactgcgtggaaaatcaacaaaaaggtgttagctgtggcgaacgtaattacaaaatggaagcactgcccggttgaggacatcccggctattgaacgtgaagagctgccaatgaaaccagaggacattgacatgaatccggaggcgctgaccgcatggaaacgtgcggcagcagcggtctatatgaaggataaagccagaaagagccgtcgtatctccctggaattcatgcttgagcaggcgaacaaattcgctaaccacaaagccatctggtttccgtataatatggattggcgtggtcgtgtttacgcggtatcgatgttcaacccgcagggtaatgacatgaccaagggtttgttgaccttggccaaaggtaaaccgattggcaaagaaggttactattggttgaagatccacggtgcgaactgcgcaggggtggataaggtaccgttcccggaacgtattaaattcatcgaggaaaaccacgaaaacattatggcgtgcgcaaagagcccgctggaaaacacgtggtgggcagagcaggacagtccattctgcttcttggcgttctgtttcgaatatgcaggtgtccagcaccacggcctgagctataactgcagcctgccgctggcctttgatggttcttgtagcggtattcaacactttagcgccatgctgcgcgatgaggttggtggcagagcagtgaatctgctgccaagcgaaaccgtgcaagatatctatggcattgtggctaagaaggttaatgaaatcctgcaagcagacgcgattaacggcacggacaacgaggttgtcaccgtgaccgatgaaaacaccggtgagatctcggagaaagtgaaactgggcaccaaagccttggctggccaatggctggcatacggcgttactcgctccgtgaccaagcgttcggtgatgacccttgcttacggcagcaaagagtttggtttccgccaacaggttctggaggatactatccaaccggccatcgactctggtaaaggcctgatgttcacgcagccgaatcaggcagcgggctatatggcgaagctgatttgggaatcggttagcgttaccgttgttgcagcggtggaggctatgaactggctgaaatctgcggcgaagctgttagctgcggaggtgaaggacaagaagacgggcgaaatcctgcgtaagcgctgcgcagtgcattgggttacgccggatggttttccggtatggcaggagtacaaaaagcctattcagacccgtctgaacctgatgtttctgggtcaatttcgtctgcagccgacgatcaacaccaataaggactccgagatcgacgcgcacaaacaggagtctggcatcgcacccaatttcgttcactcacaggacggttcccatctgcgtaagaccgtcgtgtgggcacacgagaagtatggcattgagtcgtttgcattgatccacgattcctttggtaccatcccggcggacgctgcgaacctgtttaaagcggttcgcgaaaccatggttgacacctatgaaagttgcgatgttctggcagacttttatgatcagttcgccgaccaactgcatgagtcccagctggataaaatgccggcgttaccggcgaagggcaacttaaatctccgcgacatcctggaatctgatttcgccttcgcgtaa

SEQ ID NO: 40 - DNA, 2652 bp, synthetic construct
  source 1..2652: mol_type = other DNA
atgaatacaattaacatagctaaaaatgatttcagcgatattgaactggctgcgatcccgtttaataccttggcggaccattatggtgagcgtctggcgcgtgagcaacttgctctggagcacgaatcctacgagatgggtgaagcgcgtttccggaagatgttcgagcgccagcttaaggctggcgaggtggcggataacgctgctgcgaagccgttgattacgaccctgctgccgaaaatgattgcgcgtattaacgattggttcgaggaagtgaaagcaaagcgtggtaaacgtccaaccgcattccagtttctgcaagagatcaagccggaggcggtggcatacattacgatcaaaaccactctcgcatgtctcaccagcgcggataatactacggtccaagcggtggccagcgcgattggccgcgcgattgaggacgaagcgcgttttggtcgcattcgtgacctggaagcgaaacattttaagaagaacgttgaagaacaattgaataaacgcgtgggccacgtttacaagaaagcgttcatgcaagtcgttgaagctgatatgctgagcaaaggcctgttaggtggtgaagcatggagcagctggcataaggaggactcaattcacgtcggcgtgcggtgcattgaaatgctgatcgaatcgaccggtatggttagcctgcatcgccaaaacgccggcgtggtgggtcaagatagcgaaacgattgaactggcgccagagtacgcggaagctatcgctaccagagccggcgcattggcggggatcagcccgatgttccagccgtgtgttgtaccaccgaagccgtggaccggtatcaccggtggaggttactgggcgaatggtagacgtccgttggcgttggttcgtacccatagcaaaaaggctctgatgcgttatgaagacgtttacatgccggaagtgtacaaagccatcaacatcgcgcagaacactgcgtggaaaatcaacaaaaaggtgttagctgtggcgaacgtaattacaaaatggaagcactgcccggttgaggacatcccggctattgaacgtgaagagctgccaatgaaaccagaggacattgacatgaatccggaggcgctgaccgcatggaaacgtgcggcagcagcggtctattggaaggataaagccagaaagagccgtcgtatctccctggaattcatgcttgagcaggcgaacaaattcgctaaccacaaagccatctggtttccgtataatatggattggcgtggtcgtgtttacgcggtatcgatgttcaacccgcagggtactgacatgaccaagggtttgttgaccttggccaaaggtaaaccgattggcaaagaaggttactattggttgaagatccacggtgcgaactgcgcaggggtggataaggtaccgttcccggaacgtattaaattcatcgaggaaaaccacgaaaacattatggcgtgcgcaaagagcccgctggaaaacacgtggtgggcagagcaggacagtccattctgcttcttggcgttctgtttcgaatatgcaggtgtccagcaccacggcctgagctataactgcagcctgccgctggcctttgatggttcttgtagcggtattcaacactttagcgccatgctgcgcgatgaggttggtggcagagcagtgaatctgctgccaagcgaaaccgtgcaagatatctatggcattgtggctaagaaggttaatgaaatcctgcaagcagacgcgattaacggcacggacaacgaggttgtcaccgtgaccgatgaaaacaccggtgagatctcggagaaagtgaaactgggcaccaaagccttggctggccaatggctggcatacggcgttactcgctccgtgaccaagcgttcggtgatgacccttgcttacggcagcaaagagtttggtttccgccaacaggttctggaggatactatccaaccggccatcgactctggtaaaggcctgatgttcacgcagccgaatcaggcagcgggctatatggcgaagctgatttgggaatcggttagcgttaccgttgttgcagcggtggaggctatgaactggctgaaatctgcggcgaagctgttagctgcggaggtgaaggacaagaagacgggcgaaatcctgcgtaagcgctgcgcagtgcattgggttacgccggatggttttccggtatggcaggagtacaaaaagcctattcagacccgtctgaacctgatgtttctgggtcaatttcgtctgcagccgacgatcaacaccaataaggactccgagatcgacgcgcacaaacaggagtctggcatcgcacccaatttcgttcactcacaggacggttcccatctgcgtaagaccgtcgtgtgggcacacgagaagtatggcattgagtcgtttgcattgatccacgattcctttggtaccatcccggcggacgctgcgaacctgtttaaagcggttcgcgaaaccatggttgacacctatgaaagttgcgatgttctggcagacttttatgatcagttcgccgaccaactgcatgagtcccagctggataaaatgccggcgttaccggcgaagggcaacttaaatctccgcgacatcctggaatctgatttcgccttcgcgtaa

SEQ ID NO: 41 - DNA, 2649 bp, synthetic construct
  source 1..2649: mol_type = other DNA
atgaatacaattaacatagctaaaaatgatttcagcgatattgaactggctgcgatcccgtttaataccttggcggaccattatggtgagcgtctggcgcgtgagcaacttgctctggagcacgaatcctacgagatgggtgaagcgcgtttccggaagatgttcgagcgccagcttaaggctggcgaggtggcggataacgctgctgcgaagccgttgattacgaccctgctgccgaaaatgattgcgcgtattaacgattggttcgaggaagtgaaagcaaagcgtggtaaacgtccaaccgcattccagtttctgcaagagatcaagccggaggcggtggcatacattacgatcaaaaccactctcgcatgtctcaccagcgcggataatactacggtccaagcggtggccagcgcgattggccgcgcgattgaggacgaagcgcgttttggtcgcattcgtgacctggaagcgaaacattttaagaagaacgttgaagaacaattgaatcgcgtgggccacgtttacaagaaagcgttcatgcaagtcgttgaagctgatatgctgagcaaaggcctgttaggtggtgaagcatggagcagctggcataaggaggactcaattcacgtcggcgtgcggtgcattgaaatgctgatcgaatcgaccggtatggttagcctgcatcgccaaaacgccggcgtggtgggtcaagatagcgaaacgattgaactggcgccagagtacgcggaagctatcgctaccagagccggcgcattggcggggatcagcccgatgttccagccgtgtgttgtaccaccgaagccgtggaccggtatcaccggtggaggttactgggcgaatggtagacgtccgttggcgttggttcgtacccatagcaaaaaggctctgatgcgttatgaagacgtttacatgccggaagtgtacaaagccatcaacatcgcgcagaacactgcgtggaaaatcaacaaaaaggtgttagctgtggcgaacgtaattacaaaatggaagcactgcccggttgaggacatcccggctattgaacgtgaagagctgccaatgaaaccagaggacattgacatgaatccggaggcgctgaccgcatggaaacgtgcggcagcagcggtctatattaaggataaagccagaaagagccgtcgtatctccctggaattcatgcttgagcaggcgaacaaattcgctaaccacaaagccatctggtttccgtataatatggattggcgtggtcgtgtttacgcggtatcgatgttcaacccgcagggtaatgacatgaccaagggtttgttgaccttggccaaaggtaaaccgattggcaaagaaggttactattggttgaagatccacggtgcgaactgcgcaggggtggataaggtaccgttcccggaacgtattaaattcatcgaggaaaaccacgaaaacattatggcgtgcgcaaagagcccgctggaaaacacgtggtgggcagagcaggacagtccattctgcttcttggcgttctgtttcgaatatgcaggtgtccagcaccacggcctgagctataactgcagcctgccgctggcctttgatggttcttgtagcggtattcaacactttagcgccatgctgcgcgatgaggttggtggcagagcagtgaatctgctgccaagcgaaaccgtgcaagatatctatggcattgtggctaagaaggttaatgaaatcctgcaagcagacgcgattaacggcacggacaacgaggttgtcaccgtgaccgatgaaaacaccggtgagatctcggagaaagtgaaactgggcaccaaagccttggctggccaatggctggcatacggcgttactcgctccgtgaccaagcgttcggtgatgacccttgcttacggcagcaaagagtttggtttccgccaacaggttctggaggatactatccaaccggccatcgactctggtaaaggcctgatgttcacgcagccgaatcaggcagcgggctatatggcgaagctgatttgggaatcggttagcgttaccgttgttgcagcggtggaggctatgaactggctgaaatctgcggcgaagctgttagctgcggaggtgaaggacaagaagacgggcgaaatcctgcgtaagcgctgcgcagtgcattgggttacgccggatggttttccggtatggcaggagtacaaaaagcctattcagacccgtctgaacctgatgtttctgggtcaatttcgtctgcagccgacgatcaacaccaataaggactccgagatcgacgcgcacaaacaggagtctggcatcgcacccaatttcgttcactcacaggacggttcccatctgcgtaagaccgtcgtgtgggcacacgagaagtatggcattgagtcgtttgcattgatccacgattcctttggtaccatcccggcggacgctgcgaacctgtttaaagcggttcgcgaaaccatggttgacacctatgaaagttgcgatgttctggcagacttttatgatcagttcgccgaccaactgcatgagtcccagctggataaaatgccggcgttaccggcgaagggcaacttaaatctccgcgacatcctggaatctgatttcgccttcgcgtaa

SEQ ID NO: 42 - DNA, 2652 bp, synthetic construct
  source 1..2652: mol_type = other DNA
atgaatacaattaacatagctaaaaatgatttcagcgatattgaactggctgcgatcccgtttaataccttggcggaccattatggtgagcgtctggcgcgtgagcaacttgctctggagcacgaatcctacgagatgggtgaagcgcgtttccggaagatgttcgagcgccagcttaaggctggcgaggtggcggataacgctgctgcgaagccgttgattacgaccctgctgccgaaaatgattgcgcgtattaacgattggttcgaggaagtgaaagcaaagcgtggtaaacgtccaaccgcattccagtttctgcaagagatcaagccggaggcggtggcatacattacgatcaaaaccactctcgcatgtctcaccagcgcggataatactacggtccaagcggtggccagcgcgattggccgcgcgattgaggacgaagcgcgttttggtcgcattcgtgacctggaagcgaaacattttaagaagaacgttgaagaacaattgaataaacgcgtgggccacgttgataagaaagcgttcatgcaagtcgttgaagctgatatgctgagcaaaggcctgttaggtggtgaagcatggagcagctggcataaggaggactcaattcacgtcggcgtgcggtgcattgaaatgctgatcgaatcgaccggtatggttagcctgcatcgccaaaacgccggcgtggtgggtcaagatagcgaaacgattgaactggcgccagagtacgcggaagctatcgctaccagagccggcgcattggcggggatcagcccgatgttccagccgtgtgttgtaccaccgaagccgtggaccggtatcaccggtggaggttactgggcgaatggtagacgtccgttggcgttggttcgtacccatagcaaaaaggctctgatgcgttatgaagacgtttacatgccggaagtgtacaaagccatcaacatcgcgcagaacactgcgtggaaaatcaacaaaaaggtgttagctgtggcgaacgtaattacaaaatggaagcactgcccggttgaggacatcccggctattgaacgtgaagagctgccaatgaaaccagaggacattgacatgaatccggaggcgctgaccgcatggaaacgtgcggcagcagcggtctattttaaggataaagccagaaagagccgtcgtatctccctggaattcatgcttgagcaggcgaacaaattcgctaaccacaaagccatctggtttccgtataatatggattggcgtggtcgtgtttacgcggtatcgatgttcaacccgcagggtaatgacatgaccaagggtttgttgaccttggccaaaggtaaaccgattggcaaagaaggttactattggttgaagatccacggtgcgaactgcgcaggggtggataaggtaccgttcccggaacgtattaaattcatcgaggaaaaccacgaaaacattatggcgtgcgcaaagagcccgctggaaaacacgtggtgggcagagcaggacagtccattctgcttcttggcgttctgtttcgaatatgcaggtgtccagcaccacggcctgagctataactgcagcctgccgctggcctttgatggttcttgtagcggtattcaacactttagcgccatgctgcgcgatgaggttggtggcagagcagtgaatctgctgccaagcgaaaccgtgcaagatatctatggcattgtggctaagaaggttaatgaaatcctgcaagcagacgcgattaacggcacggacaacgaggttgtcaccgtgaccgatgaaaacaccggtgagatctcggagaaagtgaaactgggcaccaaagccttggctggccaatggctggcatacggcgttactcgctccgtgaccaagcgttcggtgatgacccttgcttacggcagcaaagagtttggtttccgccaacaggttctggaggatactatccaaccggccatcgactctggtaaaggcctgatgttcacgcagccgaatcaggcagcgggctatatggcgaagctgatttgggaatcggttagcgttaccgttgttgcagcggtggaggctatgaactggctgaaatctgcggcgaagctgttagctgcggaggtgaaggacaagaagacgggcgaaatcctgcgtaagcgctgcgcagtgcattgggttacgccggatggttttccggtatggcaggagtacaaaaagcctattcagacccgtctgaacctgatgtttctgggtcaatttcgtctgcagccgacgatcaacaccaataaggactccgagatcgacgcgcacaaacaggagtctggcatcgcacccaatttcgttcactcacaggacggttcccatctgcgtaagaccgtcgtgtgggcacacgagaagtatggcattgagtcgtttgcattgatccacgattcctttggtaccatcccggcggacgctgcgaacctgtttaaagcggttcgcgaaaccatggttgacacctatgaaagttgcgatgttctggcagacttttatgatcagttcgccgaccaactgcatgagtcccagctggataaaatgccggcgttaccggcgaagggcaacttaaatctccgcgacatcctggaatctgatttcgccttcgcgtaa

SEQ ID NO: 43 - DNA, 2652 bp, synthetic construct
  source 1..2652: mol_type = other DNA
atgaatacaattaacatagctaaaaatgatttcagcgatattgaactggctgcgatcccgtttaataccttggcggaccattatggtgagcgtctggcgcgtgagcaacttgctctggagcacgaatcctacgagatgggtgaagcgcgtttccggaagatgttcgagcgccagcttaaggctggcgaggtggcggataacgctgctgcgaagccgttgattacgaccctgctgccgaaaatgattgcgcgtattaacgattggttcgaggaagtgaaagcaaagcgtggtaaacgtccaaccgcattccagtttctgcaagagatcaagccggaggcggtggcatacattacgatcaaaaccactctcgcatgtctcaccagcgcggataatactacggtccaagcggtggccagcgcgattggccgcgcgattgaggacgaagcgcgttttggtcgcattcgtgacctggaagcgaaacattttaagaagaacgttgaagaacaattgaataaacgcgtgggccacgtttacaagaaagcgttcatgcaagtcgttgaagctgatatgctgagcaaaggcctgttaggtggtgaagcatggagcagctggcataaggaggactcaattcacgtcggcgtgcggtgcattgaaatgctgatcgaatcgaccggtatggttagcctgcatcgccaaaacgccggcgtggtgggtcaagatagcgaaacgattgaactggcgccagagtacgcggaagctatcgctaccagagccggcgcattggcggggatcagcccgatgttccagccgtgtgttgtaccaccgaagccgtggaccggtatcaccggtggaggttactgggcgaatggtagacgtccgttggcgttggttcgtacccatagcaaaaaggctctgatgcgttatgaagacgtttacatgccggaagtgtacaaagccatcaacatcgcgcagaacactgcgtggaaaatcaacaaaaaggtgttagctgtggcgaacgtaattacaaaatggaagcactgcccggttgaggacatcccggctattgaacgtgaagagctgccaatgaaaccagaggacattgacatgaatccggaggcgctgaccgcatggaaacgtgcggcagcagcggtctatcgtaagaaaaaagccagaaagagccgtcgtatctccctggaattcatgcttgagcaggcgaacaaattcgctaaccacaaagccatctggtttccgtataatatggattggcgtggtcgtgtttacgcggtatcgatgttcaacccgcagggtaatcctatgaccaagggtttgttgaccttggccaaaggtaaaccgattggcaaagaaggttactattggttgaagatccacggtgcgaactgcgcaggggtggataaggtaccgttcccggaacgtattaaattcatcgaggaaaaccacgaaaacattatggcgtgcgcaaagagcccgctggaaaacacgtggtgggcagagcaggacagtccattctgcttcttggcgttctgtttcgaatatgcaggtgtccagcaccacggcctgagctataactgcagcctgccgctggcctttgatggttcttgtagcggtattcaacactttagcgccatgctgcgcgatgaggttggtggcagagcagtgaatctgctgccaagcgaaaccgtgcaagatatctatggcattgtggctaagaaggttaatgaaatcctgcaagcagacgcgattaacggcacggacaacgaggttgtcaccgtgaccgatgaaaacaccggtgagatctcggagaaagtgaaactgggcaccaaagccttggctggccaatggctggcatacggcgttactcgctccgtgaccaagcgttcggtgatgacccttgcttacggcagcaaagagtttggtttccgccaacaggttctggaggatactatccaaccggccatcgactctggtaaaggcctgatgttcacgcagccgaatcaggcagcgggctatatggcgaagctgatttgggaatcggttagcgttaccgttgttgcagcggtggaggctatgaactggctgaaatctgcggcgaagctgttagctgcggaggtgaaggacaagaagacgggcgaaatcctgcgtaagcgctgcgcagtgcattgggttacgccggatggttttccggtatggcaggagtacaaaaagcctattcagacccgtctgaacctgatgtttctgggtcaatttcgtctgcagccgacgatcaacaccaataaggactccgagatcgacgcgcacaaacaggagtctggcatcgcacccaatttcgttcactcacaggacggttcccatctgcgtaagaccgtcgtgtgggcacacgagaagtatggcattgagtcgtttgcattgatccacgattcctttggtaccatcccggcggacgctgcgaacctgtttaaagcggttcgcgaaaccatggttgacacctatgaaagttgcgatgttctggcagacttttatgatcagttcgccgaccaactgcatgagtcccagctggataaaatgccggcgttaccggcgaagggcaacttaaatctccgcgacatcctggaatctgatttcgccttcgcgtaa

SEQ ID NO: 44 - DNA, 2652 bp, synthetic construct
  source 1..2652: mol_type = other DNA
atgaatacaattaacatagctaaaaatgatttcagcgatattgaactggctgcgatcccgtttaataccttggcggaccattatggtgagcgtctggcgcgtgagcaacttgctctggagcacgaatcctacgagatgggtgaagcgcgtttccggaagatgttcgagcgccagcttaaggctggcgaggtggcggataacgctgctgcgaagccgttgattacgaccctgctgccgaaaatgattgcgcgtattaacgattggttcgaggaagtgaaagcaaagcgtggtaaacgtccaaccgcattccagtttctgcaagagatcaagccggaggcggtggcatacattacgatcaaaaccactctcgcatgtctcaccagcgcggataatactacggtccaagcggtggccagcgcgattggccgcgcgattgaggacgaagcgcgttttggtcgcattcgtgacctggaagcgaaacattttaagaagaacgttgaagaacaattgaataaacgcgtgggccacgtttacaagaaagcgttcatgcaagtcgttgaagctgatatgctgagcaaaggcctgttaggtggtgaagcatggagcagctggcataaggaggactcaattcacgtcggcgtgcggtgcattgaaatgctgatcgaatcgaccggtatggttagcctgcatcgccaaaacgccggcgtggtgggtcaagatagcgaaacgattgaactggcgccagagtacgcggaagctatcgctaccagagccggcgcattggcggggatcagcccgatgttccagccgtgtgttgtaccaccgaagccgtggaccggtatcaccggtggaggttactgggcgaatggtagacgtccgttggcgttggttcgtacccatagcaaaaaggctctgatgcgttatgaagacgtttacatgccggaagtgtacaaagccatcaacatcgcgcagaacactgcgtggaaaatcaacaaaaaggtgttagctgtggcgaacgtaattacaaaatggaagcactgcccggttgaggacatcccggctattgaacgtgaagagctgccaatgaaaccagaggacattgacatgaatccggaggcgctgaccgcatggaaacgtgcggcagcagcggtctattgcaaggataaagccagaaagagccgtcgtatctccctggaattcatgcttgagcaggcgaacaaattcgctaaccacaaagccatctggtttccgtataatatggattggcgtggtcgtgtttacgcggtatcgatgttcaacccgcagggtaatcctatgaccaagggtttgttgaccttggccaaaggtaaaccgattggcaaagaaggttactattggttgaagatccacggtgcgaactgcgcaggggtggataaggtaccgttcccggaacgtattaaattcatcgaggaaaaccacgaaaacattatggcgtgcgcaaagagcccgctggaaaacacgtggtgggcagagcaggacagtccattctgcttcttggcgttctgtttcgaatatgcaggtgtccagcaccacggcctgagctataactgcagcctgccgctggcctttgatggttcttgtagcggtattcaacactttagcgccatgctgcgcgatgaggttggtggcagagcagtgaatctgctgccaagcgaaaccgtgcaagatatctatggcattgtggctaagaaggttaatgaaatcctgcaagcagacgcgattaacggcacggacaacgaggttgtcaccgtgaccgatgaaaacaccggtgagatctcggagaaagtgaaactgggcaccaaagccttggctggccaatggctggcatacggcgttactcgctccgtgaccaagcgttcggtgatgacccttgcttacggcagcaaagagtttggtttccgccaacaggttctggaggatactatccaaccggccatcgactctggtaaaggcctgatgttcacgcagccgaatcaggcagcgggctatatggcgaagctgatttgggaatcggttagcgttaccgttgttgcagcggtggaggctatgaactggctgaaatctgcggcgaagctgttagctgcggaggtgaaggacaagaagacgggcgaaatcctgcgtaagcgctgcgcagtgcattgggttacgccggatggttttccggtatggcaggagtacaaaaagcctattcagacccgtctgaacctgatgtttctgggtcaatttcgtctgcagccgacgatcaacaccaataaggactccgagatcgacgcgcacaaacaggagtctggcatcgcacccaatttcgttcactcacaggacggttcccatctgcgtaagaccgtcgtgtgggcacacgagaagtatggcattgagtcgtttgcattgatccacgattcctttggtaccatcccggcggacgctgcgaacctgtttaaagcggttcgcgaaaccatggttgacacctatgaaagttgcgatgttctggcagacttttatgatcagttcgccgaccaactgcatgagtcccagctggataaaatgccggcgttaccggcgaagggcaacttaaatctccgcgacatcctggaatctgatttcgccttcgcgtaa

SEQ ID NO: 45 - DNA, 4388 bp, synthetic construct
  source 1..4388: mol_type = other DNA
taatacgactcactatagggagaaaataacaaatctcaacacaacatatacaaaacaaacgaatctcaagcaatcaagcattctacttctattgcagcaatttaaatcatttcttttaaagcaaaagcaattttctgaaaattttcaccatttacgaacgatagcagccaccatgttcgtgtttctggtgctgctgcctctggtgagctcccagtgcgtgaatctgaccacaaggacccagctgccccctgcctataccaactccttcacacggggcgtgtactatcccgacaaggtgttccggagcagcgtgctgcactccacacaggatctgtttctgcctttcttttctaacgtgacctggttccacgccatccacgtgagcggcaccaatggcacaaagaggttcgacaacccagtgctgcccttcaatgatggcgtgtacttcgcctccaccgagaagtctaatatcatccgcggctggatctttggcaccacactggacagcaagacacagtccctgctgatcgtgaacaatgccaccaacgtggtcatcaaggtgtgcgagttccagttttgtaacgatccattcctgggcgtgtactatcacaagaacaataagtcttggatggagagcgagtttcgcgtgtattcctctgccaacaattgcacatttgagtacgtgtcccagcccttcctgatggacctggagggcaagcagggcaatttcaagaacctgcgggagttcgtgtttaagaacatcgatggctacttcaaaatctactccaagcacaccccaatcaatctggtgagagacctgccacagggcttctctgccctggagccactggtggatctgcccatcggcatcaacatcacccggtttcagacactgctggccctgcacagaagctacctgacaccaggcgacagctcctctggatggaccgcaggagcagcagcctactatgtgggctatctgcagcccaggaccttcctgctgaagtacaacgagaatggcaccatcacagacgcagtggattgcgcactggaccccctgtctgagaccaagtgtacactgaagtcctttaccgtggagaagggcatctatcagacaagcaacttcagggtgcagcctaccgagtccatcgtgcgctttcccaatatcacaaacctgtgcccttttggcgaggtgttcaatgcaaccaggttcgcaagcgtgtacgcatggaataggaagcgcatctccaactgcgtggccgactattctgtgctgtacaatagcgcctccttctctacctttaagtgctacggcgtgagccccacaaagctgaatgacctgtgctttaccaacgtgtacgccgattccttcgtgatcaggggcgacgaggtgcgccagatcgcaccaggacagacaggcaagatcgcagactacaactataagctgcctgacgatttcaccggctgcgtgatcgcctggaacagcaacaatctggatagcaaagtgggcggcaactacaattatctgtaccggctgtttagaaagtctaacctgaagccattcgagagggacatctccacagaaatctaccaggccggctctaccccctgcaatggcgtggagggctttaactgttatttccctctgcagagctacggcttccagccaacaaatggcgtgggctatcagccctaccgcgtggtggtgctgtcttttgagctgctgcacgcccctgcaacagtgtgcggaccaaagaagtccaccaatctggtgaagaacaagtgcgtgaacttcaacttcaacggactgaccggcacaggcgtgctgaccgagtccaacaagaagttcctgccttttcagcagttcggcagggacatcgcagataccacagacgccgtgcgcgaccctcagaccctggagatcctggatatcacaccatgctccttcggcggcgtgtctgtgatcacaccaggcaccaatacaagcaaccaggtggccgtgctgtatcaggacgtgaactgtaccgaggtgcccgtggcaatccacgcagatcagctgacccctacatggcgggtgtactctaccggcagcaacgtgttccagacaagagccggatgcctgatcggagcagagcacgtgaacaatagctatgagtgcgacatccctatcggcgccggcatctgtgcctcctaccagacccagacaaactccccaaggagagcacggtctgtggcaagccagtccatcatcgcctataccatgagcctgggcgccgagaactccgtggcctactccaacaattctatcgccatccctaccaatttcacaatctccgtgaccacagagatcctgccagtgagcatgaccaagacatccgtggactgcacaatgtatatctgtggcgattccaccgagtgctctaatctgctgctgcagtacggctctttttgtacccagctgaacagagccctgacaggcatcgccgtggagcaggacaagaatacacaggaggtgttcgcccaggtgaagcaaatctacaagaccccacccatcaaggactttggcggcttcaactttagccagatcctgcccgatcctagcaagccatccaagcggtcttttatcgaggacctgctgttcaataaggtgaccctggccgatgccggcttcatcaagcagtatggcgattgcctgggcgacatcgccgccagagacctgatctgtgcccagaagtttaacggcctgaccgtgctgcctccactgctgacagatgagatgatcgcccagtacacatctgccctgctggcaggcaccatcacaagcggatggaccttcggcgcaggagccgccctgcagatcccctttgccatgcagatggcctatcggttcaatggcatcggcgtgacccagaatgtgctgtacgagaaccagaagctgatcgccaatcagtttaactccgccatcggcaagatccaggactctctgagctccacagcaagcgccctgggcaagctgcaggatgtggtgaatcagaacgcccaggccctgaacaccctggtgaagcagctgtctagcaatttcggcgccatctcctctgtgctgaacgatatcctgagccggctggacaaggtggaggcagaggtgcagatcgaccggctgatcacaggcagactgcagtccctgcagacctacgtgacacagcagctgatcagggcagcagagatcagggcatctgccaacctggcagcaaccaagatgagcgagtgcgtgctgggccagtccaagagagtggacttttgtggcaagggctatcacctgatgagcttcccacagtccgcccctcacggagtggtgtttctgcacgtgacctacgtgccagcccaggagaagaacttcaccacagcaccagcaatctgccacgatggcaaggcacactttcctagggagggcgtgttcgtgagcaatggcacccactggtttgtgacacagcgcaacttctacgagccacagatcatcaccacagacaatacattcgtgtccggcaactgtgacgtggtcatcggcatcgtgaacaataccgtgtatgatcctctgcagccagagctggactcttttaaggaggagctggataagtacttcaagaaccacaccagccccgacgtggatctgggcgacatctctggcatcaatgccagcgtggtgaacatccagaaggagatcgacaggctgaatgaggtggccaagaatctgaacgagtccctgatcgatctgcaggagctgggcaagtatgagcagtacatcaagtggccctggtatatctggctgggcttcatcgccggcctgatcgccatcgtgatggtgaccatcatgctgtgctgtatgacaagctgctgttcctgcctgaagggctgctgttcttgtggcagctgctgtaagtttgatgaggacgatagcgagcctgtgctgaagggcgtgaagctgcactacacctgagaattcaaccagcctcaagaacacccgaatggagtctctaagctacataataccaacttacactttacaaaatgttgtcccccaaaatgtagccattcgtatctgctcctaataaaaagaaagtttcttcacattctaaccagcctcaagaacacccgaatggagtctctaagctacataataccaacttacactttacaaaatgttgtcccccaaaatgtagccattcgtatctgctcctaataaaaagaaagtttcttcacattctaagcttaaaaaaaaaaaaaaaaaaaaaaaaaaaaaaaaaaaaaaaaaaaaaaaaaaaaaaaaaaaaaaaaaaaaaaaaaaaaaaaaaaaaaaaaaaaaaaaaaaaaaaaaaaaaaaaaaaaaaaaa